European Patent Application EP 4 406 606 A2, published July 31, 2024. Title: Binder-Wirkstoff-Konjugate (ADCs) und Binder-Prodrug-Konjugate (APDCs) mit enzymatisch-spaltbaren Gruppen. Applicant: Bayer Pharma Aktiengesellschaft. Application EP. The sequence listing filed with the application follows.

SEQUENCE LISTING (245 sequences)

SEQ ID NO: 1 - protein, 215 aa, Homo Sapiens
DIQMTQSPSSLSASVGDRVTITCRASQSISGYLNWYQQKPGKAPKLLIYQASSLQSGVPSRFSGSGSGTDFTLTISSLQPEDFATYYCQQSYTSPFITFGQGTKVEIKRTVAAPSVFIFPPSDEQLKSGTASVVCLLNNFYPREAKVQWKVDNALQSGNSQESVTEQDSKDSTYSLSSTLTLSKADYEKHKVYACEVTHQGLSSPVTKSFNRGEC

SEQ ID NO: 2 - protein, 449 aa, Homo Sapiens
EVQLLESGGGLVQPGGSLRLSCAASGFTFSPYPMIWVRQAPGKGLEWVSYISPSGGSTHYADSVKGRFTISRDNSKNTLYLQMNSLRAEDTAVYYCARGGDTYFDYFDYWGQGTLVTVSSASTKGPSVFPLAPSSKSTSGGTAALGCLVKDYFPEPVTVSWNSGALTSGVHTFPAVLQSSGLYSLSSVVTVPSSSLGTQTYICNVNHKPSNTKVDKKVEPKSCDKTHTCPPCPAPELLGGPSVFLFPPKPKDTLMISRTPEVTCVVVDVSHEDPEVKFNWYVDGVEVHNAKTKPREEQYNSTYRVVSVLTVLHQDWLNGKEYKCKVSNKALPAPIEKTISKAKGQPREPQVYTLPPSRDELTKNQVSLTCLVKGFYPSDIAVEWESNGQPENNYKTTPPVLDSDGSFFLYSKLTVDKSRWQQGNVFSCSVMHEALHNHYTQKSLSLSPG

SEQ ID NO: 3 - protein, 11 aa, Homo Sapiens
RASQSISGYLN

SEQ ID NO: 4 - protein, 7 aa, Homo Sapiens
QASSLQS

SEQ ID NO: 5 - protein, 10 aa, Homo Sapiens
QQSYTSPFIT

SEQ ID NO: 6 - protein, 5 aa, Homo Sapiens
PYPMI

SEQ ID NO: 7 - protein, 17 aa, Homo Sapiens
YISPSGGSTHYADSVKG

SEQ ID NO: 8 - protein, 11 aa, Homo Sapiens
GGDTYFDYFDY

SEQ ID NO: 9 - protein, 108 aa, Homo Sapiens
DIQMTQSPSSLSASVGDRVTITCRASQSISGYLNWYQQKPGKAPKLLIYQASSLQSGVPSRFSGSGSGTDFTLTISSLQPEDFATYYCQQSYTSPFITFGQGTKVEIK

SEQ ID NO: 10 - protein, 121 aa, Homo Sapiens
EVQLLESGGGLVQPGGSLRLSCAASGFTFSPYPMIWVRQAPGKGLEWVSYISPSGGSTHYADSVKGRFTISRDNSKNTLYLQMNSLRAEDTAVYYCARGGDTYFDYFDYWGQGTLVTVSSA

SEQ ID NO: 11 - protein, 215 aa, Homo Sapiens
DIQMTQSPATLSASVGDRVTITCRASQSISGYLNWYQQKPGKAPKLLIYQASSLQSGVPSRFSGSGSGTDFTLTISSLQPEDFATYYCQQSYTSPFITFGPGTKVEIKRTVAAPSVFIFPPSDEQLKSGTASVVCLLNNFYPREAKVQWKVDNALQSGNSQESVTEQDSKDSTYSLSSTLTLSKADYEKHKLYACEVTHQGLSSPVTKSFNRGEC

SEQ ID NO: 12 - protein, 449 aa, Homo Sapiens
EVQLLESGGGLVQPGGSLRLSCAASGFTFSPYPMIWVRQAPGKGLEWVSYISPSGGKTHYADSVKGRFTISRDNSKNTLYLQMNSLRAEDTAVYYCARGGDTYFDYFDYWGQGTLVTVSSASTKGPSVFPLAPSSKSTSGGTAALGCLVKDYFPEPVTVSWNSGALTSGVHTFPAVLQSSGLYSLSSVVTVPSSSLGTQTYICNVNHKPSNTKVDKKVEPKSCDKTHTCPPCPAPELLGGPSVFLFPPKPKDTLMISRTPEVTCVVVDVSHEDPEVKFNWYVDGVEVHNAKTKPREEQYNSTYRVVSVLTVLHQDWLNGKEYKCKVSNKALPAPIEKTISKAKGQPREPQVYTLPPSRDELTKNQVSLTCLVKGFYPSDIAVEWESNGQPENNYKTTPPVLDSDGSFFLYSKLTVDKSRWQQGNVFSCSVMHEALHNHYTQKSLSLSPG

SEQ ID NO: 13 - protein, 11 aa, Homo Sapiens
RASQSISGYLN

SEQ ID NO: 14 - protein, 7 aa, Homo Sapiens
QASSLQS

SEQ ID NO: 15 - protein, 10 aa, Homo Sapiens
QQSYTSPFIT

SEQ ID NO: 16 - protein, 5 aa, Homo Sapiens
PYPMI

SEQ ID NO: 17 - protein, 17 aa, Homo Sapiens
YISPSGGKTHYADSVKG

SEQ ID NO: 18 - protein, 11 aa, Homo Sapiens
GGDTYFDYFDY

SEQ ID NO: 19 - protein, 108 aa, Homo Sapiens
DIQMTQSPATLSASVGDRVTITCRASQSISGYLNWYQQKPGKAPKLLIYQASSLQSGVPSRFSGSGSGTDFTLTISSLQPEDFATYYCQQSYTSPFITFGPGTKVEIK

SEQ ID NO: 20 - protein, 121 aa, Homo Sapiens
EVQLLESGGGLVQPGGSLRLSCAASGFTFSPYPMIWVRQAPGKGLEWVSYISPSGGKTHYADSVKGRFTISRDNSKNTLYLQMNSLRAEDTAVYYCARGGDTYFDYFDYWGQGTLVTVSSA

SEQ ID NO: 21 - protein, 215 aa, Homo Sapiens
DIQMTQSPSSLSASVGDRVTITCRASQSISSYLNWYQQKPGKAPKLLIYQASSLQSGVPSRFSGSGSGTDFTLTISSLQPEDFATYYCQQSYTSPFITFGQGTKVEIKRTVAAPSVFIFPPSDEQLKSGTASVVCLLNNFYPREAKVQWKVDNALQSGNSQESVTEQDSKDSTYSLSSTLTLSKADYEKHKVYACEVTHQGLSSPVTKSFNRGEC

SEQ ID NO: 22 - protein, 449 aa, Homo Sapiens
EVQLLESGGGLVQPGGSLRLSCAASGFTFSPYPMMWVRQAPGKGLEWVSYISPSGGSTHYADSVKGRFTISRDNSKNTLYLQMNSLRAEDTAVYYCARGGDTYFDYFDYWGQGTLVTVSSASTKGPSVFPLAPSSKSTSGGTAALGCLVKDYFPEPVTVSWNSGALTSGVHTFPAVLQSSGLYSLSSVVTVPSSSLGTQTYICNVNHKPSNTKVDKKVEPKSCDKTHTCPPCPAPELLGGPSVFLFPPKPKDTLMISRTPEVTCVVVDVSHEDPEVKFNWYVDGVEVHNAKTKPREEQYNSTYRVVSVLTVLHQDWLNGKEYKCKVSNKALPAPIEKTISKAKGQPREPQVYTLPPSRDELTKNQVSLTCLVKGFYPSDIAVEWESNGQPENNYKTTPPVLDSDGSFFLYSKLTVDKSRWQQGNVFSCSVMHEALHNHYTQKSLSLSPG

SEQ ID NO: 23 - protein, 11 aa, Homo Sapiens
RASQSISSYLN

SEQ ID NO: 24 - protein, 7 aa, Homo Sapiens
QASSLQS

SEQ ID NO: 25 - protein, 10 aa, Homo Sapiens
QQSYTSPFIT

SEQ ID NO: 26 - protein, 5 aa, Homo Sapiens
PYPMM

SEQ ID NO: 27 - protein, 17 aa, Homo Sapiens
YISPSGGSTHYADSVKG

SEQ ID NO: 28 - protein, 11 aa, Homo Sapiens
GGDTYFDYFDY

SEQ ID NO: 29 - protein, 108 aa, Homo Sapiens
DIQMTQSPSSLSASVGDRVTITCRASQSISSYLNWYQQKPGKAPKLLIYQASSLQSGVPSRFSGSGSGTDFTLTISSLQPEDFATYYCQQSYTSPFITFGQGTKVEIK

SEQ ID NO: 30 - protein, 121 aa, Homo Sapiens
EVQLLESGGGLVQPGGSLRLSCAASGFTFSPYPMMWVRQAPGKGLEWVSYISPSGGSTHYADSVKGRFTISRDNSKNTLYLQMNSLRAEDTAVYYCARGGDTYFDYFDYWGQGTLVTVSSA

SEQ ID NO: 31 - protein, 215 aa, Homo Sapiens
DIQMTQSPATLSASVGDRVTITCRASQSISSYLNWYQQKPGKAPKLLIYQASSLQSGVPSRFSGSGSGTDFTLTISSLQPEDFATYYCQQSYTSPFITFGPGTKVEIKRTVAAPSVFIFPPSDEQLKSGTASVVCLLNNFYPREAKVQWKVDNALQSGNSQESVTEQDSKDSTYSLSSTLTLSKADYEKHKLYACEVTHQGLSSPVTKSFNRGEC

SEQ ID NO: 32 - protein, 449 aa, Homo Sapiens
EVQLLESGGGLVQPGGSLRLSCAASGFTFSPYPMMWVRQAPGKGLEWVSYISPSGGKTHYADSVKGRFTISRDNSKNTLYLQMNSLRAEDTAVYYCARGGDTYFDYFDYWGQGTLVTVSSASTKGPSVFPLAPSSKSTSGGTAALGCLVKDYFPEPVTVSWNSGALTSGVHTFPAVLQSSGLYSLSSVVTVPSSSLGTQTYICNVNHKPSNTKVDKKVEPKSCDKTHTCPPCPAPELLGGPSVFLFPPKPKDTLMISRTPEVTCVVVDVSHEDPEVKFNWYVDGVEVHNAKTKPREEQYNSTYRVVSVLTVLHQDWLNGKEYKCKVSNKALPAPIEKTISKAKGQPREPQVYTLPPSRDELTKNQVSLTCLVKGFYPSDIAVEWESNGQPENNYKTTPPVLDSDGSFFLYSKLTVDKSRWQQGNVFSCSVMHEALHNHYTQKSLSLSPG

SEQ ID NO: 33 - protein, 11 aa, Homo Sapiens
RASQSISSYLN

SEQ ID NO: 34 - protein, 7 aa, Homo Sapiens
QASSLQS

SEQ ID NO: 35 - protein, 10 aa, Homo Sapiens
QQSYTSPFIT

SEQ ID NO: 36 - protein, 5 aa, Homo Sapiens
PYPMM

SEQ ID NO: 37 - protein, 17 aa, Homo Sapiens
YISPSGGKTHYADSVKG

SEQ ID NO: 38 - protein, 11 aa, Homo Sapiens
GGDTYFDYFDY

SEQ ID NO: 39 - protein, 108 aa, Homo Sapiens
DIQMTQSPATLSASVGDRVTITCRASQSISSYLNWYQQKPGKAPKLLIYQASSLQSGVPSRFSGSGSGTDFTLTISSLQPEDFATYYCQQSYTSPFITFGPGTKVEIK

SEQ ID NO: 40 - protein, 121 aa, Homo Sapiens
EVQLLESGGGLVQPGGSLRLSCAASGFTFSPYPMMWVRQAPGKGLEWVSYISPSGGKTHYADSVKGRFTISRDNSKNTLYLQMNSLRAEDTAVYYCARGGDTYFDYFDYWGQGTLVTVSSA

SEQ ID NO: 41 - protein, 215 aa, Homo Sapiens
DIQMTQSPSSLSASVGDRVTITCRASQSISSYLNWYQQKPGKAPKLLIYAASSLQSGVPSRFSGSGSGTDFTLTISSLQPEDFATYYCQQSYSTPGITFGQGTKVEIKRTVAAPSVFIFPPSDEQLKSGTASVVCLLNNFYPREAKVQWKVDNALQSGNSQESVTEQDSKDSTYSLSSTLTLSKADYEKHKVYACEVTHQGLSSPVTKSFNRGEC

SEQ ID NO: 42 - protein, 449 aa, Homo Sapiens; identical to SEQ ID NO: 22

SEQ ID NO: 43 - protein, 11 aa, Homo Sapiens
RASQSISSYLN

SEQ ID NO: 44 - protein, 7 aa, Homo Sapiens
AASSLQS

SEQ ID NO: 45 - protein, 10 aa, Homo Sapiens
QQSYSTPGIT

SEQ ID NO: 46 - protein, 5 aa, Homo Sapiens
PYPMM

SEQ ID NO: 47 - protein, 17 aa, Homo Sapiens
YISPSGGSTHYADSVKG

SEQ ID NO: 48 - protein, 11 aa, Homo Sapiens
GGDTYFDYFDY

SEQ ID NO: 49 - protein, 108 aa, Homo Sapiens
DIQMTQSPSSLSASVGDRVTITCRASQSISSYLNWYQQKPGKAPKLLIYAASSLQSGVPSRFSGSGSGTDFTLTISSLQPEDFATYYCQQSYSTPGITFGQGTKVEIK

SEQ ID NO: 50 - protein, 121 aa, Homo Sapiens; identical to SEQ ID NO: 30

SEQ ID NO: 51 - protein, 215 aa, Homo Sapiens
DIQMTQSPATLSASVGDRVTITCRASQSISSYLNWYQQKPGKAPKLLIYAASSLQSGVPSRFSGSGSGTDFTLTISSLQPEDFATYYCQQSYSSPGITFGPGTKVEIKRTVAAPSVFIFPPSDEQLKSGTASVVCLLNNFYPREAKVQWKVDNALQSGNSQESVTEQDSKDSTYSLSSTLTLSKADYEKHKLYACEVTHQGLSSPVTKSFNRGEC

SEQ ID NO: 52 - protein, 449 aa, Homo Sapiens; identical to SEQ ID NO: 32

SEQ ID NO: 53 - protein, 11 aa, Homo Sapiens
RASQSISSYLN

SEQ ID NO: 54 - protein, 7 aa, Homo Sapiens
AASSLQS

SEQ ID NO: 55 - protein, 10 aa, Homo Sapiens
QQSYSSPGIT

SEQ ID NO: 56 - protein, 5 aa, Homo Sapiens
PYPMM

SEQ ID NO: 57 - protein, 17 aa, Homo Sapiens
YISPSGGKTHYADSVKG

SEQ ID NO: 58 - protein, 11 aa, Homo Sapiens
GGDTYFDYFDY

SEQ ID NO: 59 - protein, 108 aa, Homo Sapiens
DIQMTQSPATLSASVGDRVTITCRASQSISSYLNWYQQKPGKAPKLLIYAASSLQSGVPSRFSGSGSGTDFTLTISSLQPEDFATYYCQQSYSSPGITFGPGTKVEIK

SEQ ID NO: 60 - protein, 121 aa, Homo Sapiens; identical to SEQ ID NO: 40

SEQ ID NO: 61 - protein, 217 aa, Homo Sapiens
AQDIQMTQSPATLSASVGDRVTITCRASQSISSYLNWYQQKPGKAPKLLIYAASSLQSGVPSRFSGSGSGTDFTLTISSLQPEDFATYYCQQSYSSPGITFGPGTKVEIKRTVAAPSVFIFPPSDEQLKSGTASVVCLLNNFYPREAKVQWKVDNALQSGNSQESVTEQDSKDSTYSLSSTLTLSKADYEKHKLYACEVTHQGLSSPVTKSFNRGEC

SEQ ID NO: 62 - protein, 449 aa, Homo Sapiens; identical to SEQ ID NO: 32

SEQ ID NO: 63 - protein, 11 aa, Homo Sapiens
RASQSISSYLN

SEQ ID NO: 64 - protein, 7 aa, Homo Sapiens
AASSLQS

SEQ ID NO: 65 - protein, 10 aa, Homo Sapiens
QQSYSSPGIT

SEQ ID NO: 66 - protein, 5 aa, Homo Sapiens
PYPMM

SEQ ID NO: 67 - protein, 17 aa, Homo Sapiens
YISPSGGKTHYADSVKG

SEQ ID NO: 68 - protein, 11 aa, Homo Sapiens
GGDTYFDYFDY

SEQ ID NO: 69 - protein, 110 aa, Homo Sapiens
AQDIQMTQSPATLSASVGDRVTITCRASQSISSYLNWYQQKPGKAPKLLIYAASSLQSGVPSRFSGSGSGTDFTLTISSLQPEDFATYYCQQSYSSPGITFGPGTKVEIK

SEQ ID NO: 70 - protein, 121 aa, Homo Sapiens; identical to SEQ ID NO: 40

SEQ ID NO: 71 - protein, 217 aa, Homo Sapiens; identical to SEQ ID NO: 61

SEQ ID NO: 72 - protein, 449 aa, Homo Sapiens
EVQLLESGGGLVQPGGSLRLSCAASGFTFSPYPMMWVRQAPGKGLEWVSYISPSGGKTHYADSVKGRFTISRDNSKNTLYLQMNSLRAEDTAVYYCARGGDGYFDYFDYWGQGTLVTVSSASTKGPSVFPLAPSSKSTSGGTAALGCLVKDYFPEPVTVSWNSGALTSGVHTFPAVLQSSGLYSLSSVVTVPSSSLGTQTYICNVNHKPSNTKVDKRVEPKSCDKTHTCPPCPAPELLGGPSVFLFPPKPKDTLMISRTPEVTCVVVDVSHEDPEVKFNWYVDGVEVHNAKTKPREEQYNSTYRVVSVLTVLHQDWLNGKEYKCKVSNKALPAPIEKTISKAKGQPREPQVYTLPPSREEMTKNQVSLTCLVKGFYPSDIAVEWESNGQPENNYKTTPPVLDSDGSFFLYSKLTVDKSRWQQGNVFSCSVMHEALHNHYTQKSLSLSPG

SEQ ID NO: 73 - protein, 11 aa, Homo Sapiens
RASQSISSYLN

SEQ ID NO: 74 - protein, 7 aa, Homo Sapiens
AASSLQS

SEQ ID NO: 75 - protein, 10 aa, Homo Sapiens
QQSYSSPGIT

SEQ ID NO: 76 - protein, 5 aa, Homo Sapiens
PYPMM

SEQ ID NO: 77 - protein, 17 aa, Homo Sapiens
YISPSGGKTHYADSVKG

SEQ ID NO: 78 - protein, 11 aa, Homo Sapiens
GGDGYFDYFDY

SEQ ID NO: 79 - protein, 110 aa, Homo Sapiens; identical to SEQ ID NO: 69

SEQ ID NO: 80 - protein, 121 aa, Homo Sapiens
EVQLLESGGGLVQPGGSLRLSCAASGFTFSPYPMMWVRQAPGKGLEWVSYISPSGGKTHYADSVKGRFTISRDNSKNTLYLQMNSLRAEDTAVYYCARGGDGYFDYFDYWGQGTLVTVSSA

SEQ ID NO: 81 - protein, 217 aa, Homo Sapiens
AQDIQMTQSPATLSASVGDRVTITCRASQSISGYLNWYQQKPGKAPKLLIYNASSLQSGVPSRFSGSGSGTDFTLTISSLQPEDFATYYCQQSYTSPFITFGPGTKVEIKRTVAAPSVFIFPPSDEQLKSGTASVVCLLNNFYPREAKVQWKVDNALQSGNSQESVTEQDSKDSTYSLSSTLTLSKADYEKHKLYACEVTHQGLSSPVTKSFNRGEC

SEQ ID NO: 82 - protein, 449 aa, Homo Sapiens; identical to SEQ ID NO: 12

SEQ ID NO: 83 - protein, 11 aa, Homo Sapiens
RASQSISGYLN

SEQ ID NO: 84 - protein, 7 aa, Homo Sapiens
NASSLQS

SEQ ID NO: 85 - protein, 10 aa, Homo Sapiens
QQSYTSPFIT

SEQ ID NO: 86 - protein, 5 aa, Homo Sapiens
PYPMI

SEQ ID NO: 87 - protein, 17 aa, Homo Sapiens
YISPSGGKTHYADSVKG

SEQ ID NO: 88 - protein, 11 aa, Homo Sapiens
GGDTYFDYFDY

SEQ ID NO: 89 - protein, 110 aa, Homo Sapiens
AQDIQMTQSPATLSASVGDRVTITCRASQSISGYLNWYQQKPGKAPKLLIYNASSLQSGVPSRFSGSGSGTDFTLTISSLQPEDFATYYCQQSYTSPFITFGPGTKVEIK

SEQ ID NO: 90 - protein, 121 aa, Homo Sapiens; identical to SEQ ID NO: 20

SEQ ID NO: 91 - protein, 217 aa, Homo Sapiens
AQDIQMTQSPATLSASVGDRVTITCRASQSISSYLNWYQQKPGKAPKLLIYNASSLQSGVPSRFSGSGSGTDFTLTISSLQPEDFATYYCQQSYTSPGITFGPGTKVEIKRTVAAPSVFIFPPSDEQLKSGTASVVCLLNNFYPREAKVQWKVDNALQSGNSQESVTEQDSKDSTYSLSSTLTLSKADYEKHKLYACEVTHQGLSSPVTKSFNRGEC

SEQ ID NO: 92 - protein, 449 aa, Homo Sapiens; identical to SEQ ID NO: 32

SEQ ID NO: 93 - protein, 11 aa, Homo Sapiens
RASQSISSYLN

SEQ ID NO: 94 - protein, 7 aa, Homo Sapiens
NASSLQS

SEQ ID NO: 95 - protein, 10 aa, Homo Sapiens
QQSYTSPGIT

SEQ ID NO: 96 - protein, 5 aa, Homo Sapiens
PYPMM

SEQ ID NO: 97 - protein, 17 aa, Homo Sapiens
YISPSGGKTHYADSVKG

SEQ ID NO: 98 - protein, 11 aa, Homo Sapiens
GGDTYFDYFDY

SEQ ID NO: 99 - protein, 110 aa, Homo Sapiens
AQDIQMTQSPATLSASVGDRVTITCRASQSISSYLNWYQQKPGKAPKLLIYNASSLQSGVPSRFSGSGSGTDFTLTISSLQPEDFATYYCQQSYTSPGITFGPGTKVEIK

SEQ ID NO: 100 - protein, 121 aa, Homo Sapiens; identical to SEQ ID NO: 40

SEQ ID NO: 101 - protein, 217 aa, Homo Sapiens
AQDIQMTQSPATLSASVGDRVTITCRASQSISGYLNWYQQKPGKAPKLLIYNASSLQSGVPSRFSGSGSGTDFTLTISSLQPEDFATYYCQQSYTSPGITFGPGTKVEIKRTVAAPSVFIFPPSDEQLKSGTASVVCLLNNFYPREAKVQWKVDNALQSGNSQESVTEQDSKDSTYSLSSTLTLSKADYEKHKLYACEVTHQGLSSPVTKSFNRGEC

SEQ ID NO: 102 - protein, 449 aa, Homo Sapiens; identical to SEQ ID NO: 32

SEQ ID NO: 103 - protein, 11 aa, Homo Sapiens
RASQSISGYLN

SEQ ID NO: 104 - protein, 7 aa, Homo Sapiens
NASSLQS

SEQ ID NO: 105 - protein, 10 aa, Homo Sapiens
QQSYTSPGIT

SEQ ID NO: 106 - protein, 5 aa, Homo Sapiens
PYPMM

SEQ ID NO: 107 - protein, 17 aa, Homo Sapiens
YISPSGGKTHYADSVKG

SEQ ID NO: 108 - protein, 11 aa, Homo Sapiens
GGDTYFDYFDY

SEQ ID NO: 109 - protein, 110 aa, Homo Sapiens
AQDIQMTQSPATLSASVGDRVTITCRASQSISGYLNWYQQKPGKAPKLLIYNASSLQSGVPSRFSGSGSGTDFTLTISSLQPEDFATYYCQQSYTSPGITFGPGTKVEIK

SEQ ID NO: 110 - protein, 121 aa, Homo Sapiens; identical to SEQ ID NO: 40

SEQ ID NO: 111 - protein, 217 aa, Homo Sapiens
AQDIQMTQSPATLSASVGDRVTITCRASQSISSYLNWYQQKPGKAPKLLIYNASSLQSGVPSRFSGSGSGTDFTLTISSLQPEDFATYYCQQSYTSPFITFGPGTKVEIKRTVAAPSVFIFPPSDEQLKSGTASVVCLLNNFYPREAKVQWKVDNALQSGNSQESVTEQDSKDSTYSLSSTLTLSKADYEKHKLYACEVTHQGLSSPVTKSFNRGEC

SEQ ID NO: 112 - protein, 449 aa, Homo Sapiens; identical to SEQ ID NO: 32

SEQ ID NO: 113 - protein, 11 aa, Homo Sapiens
RASQSISSYLN

SEQ ID NO: 114 - protein, 7 aa, Homo Sapiens
NASSLQS

SEQ ID NO: 115 - protein, 10 aa, Homo Sapiens
QQSYTSPFIT

SEQ ID NO: 116 - protein, 5 aa, Homo Sapiens
PYPMM

SEQ ID NO: 117 - protein, 17 aa, Homo Sapiens
YISPSGGKTHYADSVKG

SEQ ID NO: 118 - protein, 11 aa, Homo Sapiens
GGDTYFDYFDY

SEQ ID NO: 119 - protein, 110 aa, Homo Sapiens
AQDIQMTQSPATLSASVGDRVTITCRASQSISSYLNWYQQKPGKAPKLLIYNASSLQSGVPSRFSGSGSGTDFTLTISSLQPEDFATYYCQQSYTSPFITFGPGTKVEIK

SEQ ID NO: 120 - protein, 121 aa, Homo Sapiens; identical to SEQ ID NO: 40

SEQ ID NO: 121 - protein, 218 aa, Mus Musculus
DIVLTQSPASLAVSLGQRATISCRANKSVSTSSYSYMHWYQQKPGQPPKLLIKYASNLESGVPARFSGSGSGTDFILNIHPVEEEDAATYYCQHSRELPFTFGSGTKLEIKRADAAPTVSIFPPSSEQLTSGGASVVCFLNNFYPKDINVKWKIDGSERQNGVLNSWTDQDSKDSTYSMSSTLTLTKDEYERHNSYTCEATHKTSTSPIVKSFNRNEC

SEQ ID NO: 122 - protein, 450 aa, Mus Musculus
QVQLQQSGPEVVRPGVSVKISCKGSGYTFTDYGIHWVKQSHAKSLEWIGVISTYNGYTNYNQKFKGKATMTVDKSSSTAYMELARLTSEDSAIYYCARAYYGNLYYAMDYWGQGTSVTVSSAKTTAPSVYPLAPVCGDTTGSSVTLGCLVKGYFPEPVTLTWNSGSLSSGVHTFPAVLQSDLYTLSSSVTVTSSTWPSQSITCNVAHPASSTKVDKKIEPRGPTIKPCPPCKCPAPNLLGGPSVFIFPPKIKDVLMISLSPIVTCVVVDVSEDDPDVQISWFVNNVEVHTAQTQTHREDYNSTLRVVSALPIQHQDWMSGKEFKCKVNNKDLPAPIERTISKPKGSVRAPQVYVLPPPEEEMTKKQVTLTCMVTDFMPEDIYVEWTNNGKTELNYKNTEPVLDSDGSYFMYSKLRVEKKNWVERNSYSCSVVHEGLHNHHTTKSFSRTPG

SEQ ID NO: 123 - protein, 218 aa, Mus Musculus
DIVLTQSPASLTVSLGQRATISCRASQSVSTSSYSYMQWYQQRPGQPPKLLIKYATNLDSGVPARFSGSGSGTDFTLNIHPVEEEDAATYYCQHSWEIPYTFGGGTKLEIKRADAAPTVSIFPPSSEQLTSGGASVVCFLNNFYPKDINVKWKIDGSERQNGVLNSWTDQDSKDSTYSMSSTLTLTKDEYERHNSYTCEATHKTSTSPIVKSFNRNEC

SEQ ID NO: 124 - protein, 448 aa, Mus Musculus
EVKLEESGGGLVQPGGSMKLSCVASGFTFNNYWMSWVRQSPEKGLEWLAEIRLKSDNYATHYAESVKGKFTISRDDSKSRLYLQMNNLRAENTGIYYCTGGFADYFDYWGQGTTLTVSSAKTTAPSVYPLAPVCGDTTGSSVTLGCLVKGYFPEPVTLTWNSGSLSSGVHTFPAVLQSDLYTLSSSVTVTSSTWPSQSITCNVAHPASSTKVDKKIEPRGPTIKPCPPCKCPAPNLLGGPSVFIFPPKIKDVLMISLSPIVTCVVVDVSEDDPDVQISWFVNNVEVHTAQTQTHREDYNSTLRVVSALPIQHQDWMSGKEFKCKVNNKDLPAPIERTISKPKGSVRAPQVYVLPPPEEEMTKKQVTLTCMVTDFMPEDIYVEWTNNGKTELNYKNTEPVLDSDGSYFMYSKLRVEKKNWVERNSYSCSVVHEGLHNHHTTKSFSRTPG

SEQ ID NO: 125 - protein, 218 aa, Homo Sapiens
DIVLTQSPASLAVSLGQRATISCRASKSVSTSSYSYMHWYQQKPGQPPKLLIKYASNLESGVPARFSGSGSGTDFSLNIHPMEEDDTAMYFCQHSRELPFTFGGGTKLEIKRTVAAPSVFIFPPSDEQLKSGTASVVCLLNNFYPREAKVQWKVDNALQSGNSQESVTEQDSKDSTYSLSSTLTLSKADYEKHKVYACEVTHQGLSSPVTKSFNRGEC

SEQ ID NO: 126 - protein, 450 aa, Homo Sapiens
QVQLVQSGAEVKKPGASVKVSCKGSGYTFTDYGMHWVRQAPGQGLEWMGVISTYNGYTNYNQKFKGRVTMTVDKSTSTAYMELRSLRSDDTAVYYCARAYYGNLYYAMDYWGQGTLVTVSSASTKGPSVFPLAPSSKSTSGGTAALGCLVKDYFPEPVTVSWNSGALTSGVHTFPAVLQSSGLYSLSSVVTVPSSSLGTQTYICNVNHKPSNTKVDKKVEPKSCDKTHTCPPCPAPELLGGPSVFLFPPKPKDTLMISRTPEVTCVVVDVSHEDPEVKFNWYVDGVEVHNAKTKPREEQYNSTYRVVSVLTVLHQDWLNGKEYKCKVSNKALPAPIEKTISKAKGQPREPQVYTLPPSRDELTKNQVSLTCLVKGFYPSDIAVEWESNGQPENNYKTTPPVLDSDGSFFLYSKLTVDKSRWQQGNVFSCSVMHEALHNHYTQKSLSLSPG

SEQ ID NO: 127 - protein, 218 aa, Homo Sapiens
DIQMTQSPSSLSASVGDRVTITCRASQSVSTSSYSYMHWYQQKPGKAPKLLIKYASNLESGVPSRFSGSGSGTDFTLTISSLQPEDFATYYCQHSWEIPYTFGGGTKVEIKRTVAAPSVFIFPPSDEQLKSGTASVVCLLNNFYPREAKVQWKVDNALQSGNSQESVTEQDSKDSTYSLSSTLTLSKADYEKHKVYACEVTHQGLSSPVTKSFNRGEC

SEQ ID NO: 128 - protein, 449 aa, Homo Sapiens
QVELVESGGGLVQPGGSLRLSCAASGFTFSSYWMSWVRQAPGKGLEWVAEIRLKSDNYATHYAESVKGRFTISRDDSKNSLYLQMNSLRAEDTAVYYCTGYYADAMDYWGQGTLVTVSSASTKGPSVFPLAPSSKSTSGGTAALGCLVKDYFPEPVTVSWNSGALTSGVHTFPAVLQSSGLYSLSSVVTVPSSSLGTQTYICNVNHKPSNTKVDKKVEPKSCDKTHTCPPCPAPELLGGPSVFLFPPKPKDTLMISRTPEVTCVVVDVSHEDPEVKFNWYVDGVEVHNAKTKPREEQYNSTYRVVSVLTVLHQDWLNGKEYKCKVSNKALPAPIEKTISKAKGQPREPQVYTLPPSRDELTKNQVSLTCLVKGFYPSDIAVEWESNGQPENNYKTTPPVLDSDGSFFLYSKLTVDKSRWQQGNVFSCSVMHEALHNHYTQKSLSLSPGK

SEQ ID NO: 129 - protein, 218 aa, Mus Musculus
DIVLTQSPASLAVSLGQRATISCKASQSVSTSTYSYMQWYQQRPGQSPKLLIKYASKLDSGVPARFSGSGSGTDFTLNIHPVEEEDTATYYCQHSWELPYTFGGGTRLEIKRADAAPTVSIFPPSSEQLTSGGASVVCFLNNFYPKDINVKWKIDGSERQNGVLNSWTDQDSKDSTYSMSSTLTLTKDEYERHNSYTCEATHKTSTSPIVKSFNRNEC

SEQ ID NO: 130 - protein, 448 aa, Mus Musculus
EVKLGESGGGLVQPGGSMKLSCVASGFPFTKYWMNWVRQSPEKGLEWVAEIRLKSDNYATHYAESAKGRFTISRDDSRSSVYLQMNNLRAEDTAIYYCSPTYADTMDYWGQGTSVTVSSAKTTAPSVYPLAPVCGDTTGSSVTLGCLVKGYFPEPVTLTWNSGSLSSGVHTFPAVLQSDLYTLSSSVTVTSSTWPSQSITCNVAHPASSTKVDKKIEPRGPTIKPCPPCKCPAPNLLGGPSVFIFPPKIKDVLMISLSPIVTCVVVDVSEDDPDVQISWFVNNVEVHTAQTQTHREDYNSTLRVVSALPIQHQDWMSGKEFKCKVNNKDLPAPIERTISKPKGSVRAPQVYVLPPPEEEMTKKQVTLTCMVTDFMPEDIYVEWTNNGKTELNYKNTEPVLDSDGSYFMYSKLRVEKKNWVERNSYSCSVVHEGLHNHHTTKSFSRTPG

SEQ ID NO: 131 - protein, 218 aa, Mus Musculus
DIVLTQSPASLAVSLGQRATISCRASKSVSTSSYSYMHWYQQKPGQPPKLLIKYTSNLESGVPARFSGSGSGTDFILNIHPVEEEDAATYYCQHSRELPWTFGGGTKLEIKRADAAPTVSIFPPSSEQLTSGGASVVCFLNNFYPKDINVKWKIDGSERQNGVLNSWTDQDSKDSTYSMSSTLTLTKDEYERHNSYTCEATHKTSTSPIVKSFNRNEC

SEQ ID NO: 132 - protein, 451 aa, Mus Musculus
QVSLKESGPGILQPSQTLSLTCSFSGFSLSTSGMGVSWIRQPSGKGLEWLAHIYWDDDKRYNPSLKSRLTISKDTSRNQVFLKITSVDTADTATYYCARRGPDYYGYYPMDYWGQGTSVTVSAKTTAPSVYPLAPVCGDTTGSSVTLGCLVKGYFPEPVTLTWNSGSLSSGVHTFPAVLQSDLYTLSSSVTVTSSTWPSQSITCNVAHPASSTKVDKKIEPRGPTIKPCPPCKCPAPNLLGGPSVFIFPPKIKDVLMISLSPIVTCVVVDVSEDDPDVQISWFVNNVEVHTAQTQTHREDYNSTLRVVSALPIQHQDWMSGKEFKCKVNNKDLPAPIERTISKPKGSVRAPQVYVLPPPEEEMTKKQVTLTCMVTDFMPEDIYVEWTNNGKTELNYKNTEPVLDSDGSYFMYSKLRVEKKNWVERNSYSCSVVHEGLHNHHTTKSFSRTPG

SEQ ID NO: 133 - protein, 282 aa, Macaca fascicularis
EQAPGTAPCSHGSSWSADLDKCMDCASCRARPHSDFCLGCSAAPPAPFRLLWPRSDKTHTCPPCPAPELLGGPSVFLFPPKPKDTLMISRTPEVTCVVVDVSHEDPEVKFNWYVDGVEVHNAKTKPREEQYNSTYRVVSVLTVLHQDWLNGKEYKCKVSNKALPAPIEKTISKAKGQPREPQVYTLPPSREEMTKNQVSLTCLVKGFYPSDIAVEWESNGQPENNYKTTPPVLDSDGSFFLYSKLTVDKSRWQQGNVFSCSVMHEALHNHYTQKSLSLSPGK

SEQ ID NO: 134 - protein, 282 aa, Rattus norvegicus
EQAPGNAPCSSGSSWSADLDKCMDCASCPARPHSDFCLGCAAAPPAHFRMLWPRSDKTHTCPPCPAPELLGGPSVFLFPPKPKDTLMISRTPEVTCVVVDVSHEDPEVKFNWYVDGVEVHNAKTKPREEQYNSTYRVVSVLTVLHQDWLNGKEYKCKVSNKALPAPIEKTISKAKGQPREPQVYTLPPSREEMTKNQVSLTCLVKGFYPSDIAVEWESNGQPENNYKTTPPVLDSDGSFFLYSKLTVDKSRWQQGNVFSCSVMHEALHNHYTQKSLSLSPGK

SEQ ID NO: 135 - protein, 282 aa, Sus scrofa
ERVPGTTPCSRGSSWSADLDKCMDCASCPARPHSDFCLGCAAAPPASFRLLWPRSDKTHTCPPCPAPELLGGPSVFLFPPKPKDTLMISRTPEVTCVVVDVSHEDPEVKFNWYVDGVEVHNAKTKPREEQYNSTYRVVSVLTVLHQDWLNGKEYKCKVSNKALPAPIEKTISKAKGQPREPQVYTLPPSREEMTKNQVSLTCLVKGFYPSDIAVEWESNGQPENNYKTTPPVLDSDGSFFLYSKLTVDKSRWQQGNVFSCSVMHEALHNHYTQKSLSLSPGK

SEQ ID NO: 136 - protein, 282 aa, Canis lupus
ERVPGTTPCPRGSSWSADLDKCMDCASCRARPHSDFCLGCTAAPPAPFRLLWPRSDKTHTCPPCPAPELLGGPSVFLFPPKPKDTLMISRTPEVTCVVVDVSHEDPEVKFNWYVDGVEVHNAKTKPREEQYNSTYRVVSVLTVLHQDWLNGKEYKCKVSNKALPAPIEKTISKAKGQPREPQVYTLPPSREEMTKNQVSLTCLVKGFYPSDIAVEWESNGQPENNYKTTPPVLDSDGSFFLYSKLTVDKSRWQQGNVFSCSVMHEALHNHYTQKSLSLSPGK

SEQ ID NO: 137 - protein, 282 aa, Mus Musculus
EQAPGTSPCSSGSSWSADLDKCMDCASCPARPHSDFCLGCAAAPPAHFRLLWPRSDKTHTCPPCPAPELLGGPSVFLFPPKPKDTLMISRTPEVTCVVVDVSHEDPEVKFNWYVDGVEVHNAKTKPREEQYNSTYRVVSVLTVLHQDWLNGKEYKCKVSNKALPAPIEKTISKAKGQPREPQVYTLPPSREEMTKNQVSLTCLVKGFYPSDIAVEWESNGQPENNYKTTPPVLDSDGSFFLYSKLTVDKSRWQQGNVFSCSVMHEALHNHYTQKSLSLSPGK

SEQ ID NO: 138 - protein, 282 aa, Homo Sapiens
EQAPGTAPCSRGSSWSADLDKCMDCASCRARPHSDFCLGCAAAPPAPFRLLWPRSDKTHTCPPCPAPELLGGPSVFLFPPKPKDTLMISRTPEVTCVVVDVSHEDPEVKFNWYVDGVEVHNAKTKPREEQYNSTYRVVSVLTVLHQDWLNGKEYKCKVSNKALPAPIEKTISKAKGQPREPQVYTLPPSREEMTKNQVSLTCLVKGFYPSDIAVEWESNGQPENNYKTTPPVLDSDGSFFLYSKLTVDKSRWQQGNVFSCSVMHEALHNHYTQKSLSLSPGK

SEQ ID NO: 139 - protein, 296 aa, Homo Sapiens
EQAPGTAPCSRGSSWSADLDKCMDCASCRARPHSDFCLGCAAAPPAPFRLLWPIEGRMDPKSCDKTHTCPPCPAPELLGGPSVFLFPPKPKDTLMISRTPEVTCVVVDVSHEDPEVKFNWYVDGVEVHNAKTKPREEQYNSTYRVVSVLTVLHQDWLNGKEYKCKVSNKALPAPIEKTISKAKGQPREPQVYTLPPSREEMTKNQVSLTCLVKGFYPSDIAVEWESNGQPENNYKTTPPVLDSDGSFFLYSKLTVDKSRWQQGNVFSCSVMHEALHNHYTQKSLSLSPGKHHHHHH

SEQ ID NO: 140 - protein, 278 aa, Homo Sapiens
APCSRGSSWSADLDKCMDCASCRARPHSDFCLGCAIEGRMDPKSCDKTHTCPPCPAPELLGGPSVFLFPPKPKDTLMISRTPEVTCVVVDVSHEDPEVKFNWYVDGVEVHNAKTKPREEQYNSTYRVVSVLTVLHQDWLNGKEYKCKVSNKALPAPIEKTISKAKGQPREPQVYTLPPSREEMTKNQVSLTCLVKGFYPSDIAVEWESNGQPENNYKTTPPVLDSDGSFFLYSKLTVDKSRWQQGNVFSCSVMHEALHNHYTQKSLSLSPGKHHHHHH

SEQ ID NO: 141 - protein, 47 aa, Homo Sapiens
EQAPGTAPCSRGSSWSADLDKCMDCASCRARPHSDFCLGCAHHHHHH

SEQ ID NO: 142 - protein, 282 aa, Homo Sapiens
EQAPGTAPCSRGSSWSADLDKCMDCASCRARPHSDFCQGCAAAPPAPFRLLWPRSDKTHTCPPCPAPELLGGPSVFLFPPKPKDTLMISRTPEVTCVVVDVSHEDPEVKFNWYVDGVEVHNAKTKPREEQYNSTYRVVSVLTVLHQDWLNGKEYKCKVSNKALPAPIEKTISKAKGQPREPQVYTLPPSREEMTKNQVSLTCLVKGFYPSDIAVEWESNGQPENNYKTTPPVLDSDGSFFLYSKLTVDKSRWQQGNVFSCSVMHEALHNHYTQKSLSLSPGK

SEQ ID NO: 143 - protein, 282 aa, Homo Sapiens
EQAPGTAPCSRGSSWSADLDKCMDCASCRARPKSDFCLGCAAAPPAPFRLLWPRSDKTHTCPPCPAPELLGGPSVFLFPPKPKDTLMISRTPEVTCVVVDVSHEDPEVKFNWYVDGVEVHNAKTKPREEQYNSTYRVVSVLTVLHQDWLNGKEYKCKVSNKALPAPIEKTISKAKGQPREPQVYTLPPSREEMTKNQVSLTCLVKGFYPSDIAVEWESNGQPENNYKTTPPVLDSDGSFFLYSKLTVDKSRWQQGNVFSCSVMHEALHNHYTQKSLSLSPGK

SEQ ID NO: 144 - protein, 282 aa, Homo Sapiens
EQAPGTAPCSRGSSWSADLDKCMDCASCPARPHSDFCLGCAAAPPAPFRLLWPRSDKTHTCPPCPAPELLGGPSVFLFPPKPKDTLMISRTPEVTCVVVDVSHEDPEVKFNWYVDGVEVHNAKTKPREEQYNSTYRVVSVLTVLHQDWLNGKEYKCKVSNKALPAPIEKTISKAKGQPREPQVYTLPPSREEMTKNQVSLTCLVKGFYPSDIAVEWESNGQPENNYKTTPPVLDSDGSFFLYSKLTVDKSRWQQGNVFSCSVMHEALHNHYTQKSLSLSPGK

SEQ ID NO: 145 - protein, 282 aa, Homo Sapiens
EQAPGTAPCSRGSSWSADLDKCADCASCRARPHSDFCLGCAAAPPAPFRLLWPRSDKTHTCPPCPAPELLGGPSVFLFPPKPKDTLMISRTPEVTCVVVDVSHEDPEVKFNWYVDGVEVHNAKTKPREEQYNSTYRVVSVLTVLHQDWLNGKEYKCKVSNKALPAPIEKTISKAKGQPREPQVYTLPPSREEMTKNQVSLTCLVKGFYPSDIAVEWESNGQPENNYKTTPPVLDSDGSFFLYSKLTVDKSRWQQGNVFSCSVMHEALHNHYTQKSLSLSPGK

SEQ ID NO: 146 - protein, 282 aa, Homo Sapiens
EQAPGTAPCSRGSSASADLDKCMDCASCRARPHSDFCLGCAAAPPAPFRLLWPRSDKTHTCPPCPAPELLGGPSVFLFPPKPKDTLMISRTPEVTCVVVDVSHEDPEVKFNWYVDGVEVHNAKTKPREEQYNSTYRVVSVLTVLHQDWLNGKEYKCKVSNKALPAPIEKTISKAKGQPREPQVYTLPPSREEMTKNQVSLTCLVKGFYPSDIAVEWESNGQPENNYKTTPPVLDSDGSFFLYSKLTVDKSRWQQGNVFSCSVMHEALHNHYTQKSLSLSPGK

SEQ ID NO: 147 - protein, 282 aa, Homo Sapiens
EQAPGTAPCSRGRSWSADLDKCMDCASCRARPHSDFCLGCAAAPPAPFRLLWPRSDKTHTCPPCPAPELLGGPSVFLFPPKPKDTLMISRTPEVTCVVVDVSHEDPEVKFNWYVDGVEVHNAKTKPREEQYNSTYRVVSVLTVLHQDWLNGKEYKCKVSNKALPAPIEKTISKAKGQPREPQVYTLPPSREEMTKNQVSLTCLVKGFYPSDIAVEWESNGQPENNYKTTPPVLDSDGSFFLYSKLTVDKSRWQQGNVFSCSVMHEALHNHYTQKSLSLSPGK

SEQ ID NO: 148 - protein, 282 aa, Homo Sapiens
EQAPGQAPCSRGSSWSADLDKCMDCASCRARPHSDFCLGCAAAPPAPFRLLWPRSDKTHTCPPCPAPELLGGPSVFLFPPKPKDTLMISRTPEVTCVVVDVSHEDPEVKFNWYVDGVEVHNAKTKPREEQYNSTYRVVSVLTVLHQDWLNGKEYKCKVSNKALPAPIEKTISKAKGQPREPQVYTLPPSREEMTKNQVSLTCLVKGFYPSDIAVEWESNGQPENNYKTTPPVLDSDGSFFLYSKLTVDKSRWQQGNVFSCSVMHEALHNHYTQKSLSLSPGK

SEQ ID NO: 149 - protein, 278 aa, Homo Sapiens
APCSRGSSWSADLDKCMDCASCRARPHSDFCAGCAIEGRMDPKSCDKTHTCPPCPAPELLGGPSVFLFPPKPKDTLMISRTPEVTCVVVDVSHEDPEVKFNWYVDGVEVHNAKTKPREEQYNSTYRVVSVLTVLHQDWLNGKEYKCKVSNKALPAPIEKTISKAKGQPREPQVYTLPPSREEMTKNQVSLTCLVKGFYPSDIAVEWESNGQPENNYKTTPPVLDSDGSFFLYSKLTVDKSRWQQGNVFSCSVMHEALHNHYTQKSLSLSPGKHHHHHH

SEQ ID NO: 150 - protein, 278 aa, Homo Sapiens
APCSRGSSWSADLDKCMDCASCRARPHSDACLGCAIEGRMDPKSCDKTHTCPPCPAPELLGGPSVFLFPPKPKDTLMISRTPEVTCVVVDVSHEDPEVKFNWYVDGVEVHNAKTKPREEQYNSTYRVVSVLTVLHQDWLNGKEYKCKVSNKALPAPIEKTISKAKGQPREPQVYTLPPSREEMTKNQVSLTCLVKGFYPSDIAVEWESNGQPENNYKTTPPVLDSDGSFFLYSKLTVDKSRWQQGNVFSCSVMHEALHNHYTQKSLSLSPGKHHHHHH

SEQ ID NO: 151 - protein, 278 aa, Homo Sapiens
APCSRGSSWSADLDKCMDCASCRARPHSAFCLGCAIEGRMDPKSCDKTHTCPPCPAPELLGGPSVFLFPPKPKDTLMISRTPEVTCVVVDVSHEDPEVKFNWYVDGVEVHNAKTKPREEQYNSTYRVVSVLTVLHQDWLNGKEYKCKVSNKALPAPIEKTISKAKGQPREPQVYTLPPSREEMTKNQVSLTCLVKGFYPSDIAVEWESNGQPENNYKTTPPVLDSDGSFFLYSKLTVDKSRWQQGNVFSCSVMHEALHNHYTQKSLSLSPGKHHHHHH

SEQ ID NO: 152 - protein, 278 aa, Homo Sapiens
APCSRGSSWSADLDKCMDCASCRARPHADFCLGCAIEGRMDPKSCDKTHTCPPCPAPELLGGPSVFLFPPKPKDTLMISRTPEVTCVVVDVSHEDPEVKFNWYVDGVEVHNAKTKPREEQYNSTYRVVSVLTVLHQDWLNGKEYKCKVSNKALPAPIEKTISKAKGQPREPQVYTLPPSREEMTKNQVSLTCLVKGFYPSDIAVEWESNGQPENNYKTTPPVLDSDGSFFLYSKLTVDKSRWQQGNVFSCSVMHEALHNHYTQKSLSLSPGKHHHHHH

SEQ ID NO: 153 - protein, 278 aa, Homo Sapiens
APCSRGSSWSADLDKCMDCASCRARPASDFCLGCAIEGRMDPKSCDKTHTCPPCPAPELLGGPSVFLFPPKPKDTLMISRTPEVTCVVVDVSHEDPEVKFNWYVDGVEVHNAKTKPREEQYNSTYRVVSVLTVLHQDWLNGKEYKCKVSNKALPAPIEKTISKAKGQPREPQVYTLPPSREEMTKNQVSLTCLVKGFYPSDIAVEWESNGQPENNYKTTPPVLDSDGSFFLYSKLTVDKSRWQQGNVFSCSVMHEALHNHYTQKSLSLSPGKHHHHHH

SEQ ID NO: 154 - protein, 278 aa, Homo Sapiens
APCSRGSSWSADLDKCMDCASCRARAHSDFCLGCAIEGRMDPKSCDKTHTCPPCPAPELLGGPSVFLFPPKPKDTLMISRTPEVTCVVVDVSHEDPEVKFNWYVDGVEVHNAKTKPREEQYNSTYRVVSVLTVLHQDWLNGKEYKCKVSNKALPAPIEKTISKAKGQPREPQVYTLPPSREEMTKNQVSLTCLVKGFYPSDIAVEWESNGQPENNYKTTPPVLDSDGSFFLYSKLTVDKSRWQQGNVFSCSVMHEALHNHYTQKSLSLSPGKHHHHHH

SEQ ID NO: 155 - protein, 278 aa, Homo Sapiens
APCSRGSSWSADLDKCMDCASCRAAPHSDFCLGCAIEGRMDPKSCDKTHTCPPCPAPELLGGPSVFLFPPKPKDTLMISRTPEVTCVVVDVSHEDPEVKFNWYVDGVEVHNAKTKPREEQYNSTYRVVSVLTVLHQDWLNGKEYKCKVSNKALPAPIEKTISKAKGQPREPQVYTLPPSREEMTKNQVSLTCLVKGFYPSDIAVEWESNGQPENNYKTTPPVLDSDGSFFLYSKLTVDKSRWQQGNVFSCSVMHEALHNHYTQKSLSLSPGKHHHHHH

SEQ ID NO: 156 - protein, 240 aa, Homo Sapiens
APCSRGSSWSADLDKCMDCASCAARPHSDFCLGCAIEGRMDPKSCDKTHTCPPCPAPELLGGPSVFLFPPKPKDTLMISRTPEVTCVVVDVSHEDPEVKFNWYVDGVEVHNAKTKPREEQYNSTYRVVSVLTVLHQDWLNGKEYKCKVSNKALPAPIEKTISKAKGQPREPQVYTLPPSREEMTKNQVSLTCLVKGFYPSDIAVEWESNGQPENNYKTTPPVLDSDGSFFLYSKLTVDKS

SEQ ID NO: 157 - protein, 278 aa, Homo Sapiens
APCSRGSSWSADLDKCMDCAACRARPHSDFCLGCAIEGRMDPKSCDKTHTCPPCPAPELLGGPSVFLFPPKPKDTLMISRTPEVTCVVVDVSHEDPEVKFNWYVDGVEVHNAKTKPREEQYNSTYRVVSVLTVLHQDWLNGKEYKCKVSNKALPAPIEKTISKAKGQPREPQVYTLPPSREEMTKNQVSLTCLVKGFYPSDIAVEWESNGQPENNYKTTPPVLDSDGSFFLYSKLTVDKSRWQQGNVFSCSVMHEALHNHYTQKSLSLSPGKHHHHHH

SEQ ID NO: 158 - protein, 278 aa, Homo Sapiens
APCSRGSSWSADLDKCMACASCRARPHSDFCLGCAIEGRMDPKSCDKTHTCPPCPAPELLGGPSVFLFPPKPKDTLMISRTPEVTCVVVDVSHEDPEVKFNWYVDGVEVHNAKTKPREEQYNSTYRVVSVLTVLHQDWLNGKEYKCKVSNKALPAPIEKTISKAKGQPREPQVYTLPPSREEMTKNQVSLTCLVKGFYPSDIAVEWESNGQPENNYKTTPPVLDSDGSFFLYSKLTVDKSRWQQGNVFSCSVMHEALHNHYTQKSLSLSPGKHHHHHH

SEQ ID NO: 159 - protein, 278 aa, Homo Sapiens
APCSRGSSWSADLDACMDCASCRARPHSDFCLGCAIEGRMDPKSCDKTHTCPPCPAPELLGGPSVFLFPPKPKDTLMISRTPEVTCVVVDVSHEDPEVKFNWYVDGVEVHNAKTKPREEQYNSTYRVVSVLTVLHQDWLNGKEYKCKVSNKALPAPIEKTISKAKGQPREPQVYTLPPSREEMTKNQVSLTCLVKGFYPSDIAVEWESNGQPENNYKTTPPVLDSDGSFFLYSKLTVDKSRWQQGNVFSCSVMHEALHNHYTQKSLSLSPGKHHHHHH

SEQ ID NO: 160 - protein, 278 aa, Homo Sapiens
APCSRGSSWSADLAKCMDCASCRARPHSDFCLGCAIEGRMDPKSCDKTHTCPPCPAPELLGGPSVFLFPPKPKDTLMISRTPEVTCVVVDVSHEDPEVKFNWYVDGVEVHNAKTKPREEQYNSTYRVVSVLTVLHQDWLNGKEYKCKVSNKALPAPIEKTISKAKGQPREPQVYTLPPSREEMTKNQVSLTCLVKGFYPSDIAVEWESNGQPENNYKTTPPVLDSDGSFFLYSKLTVDKSRWQQGNVFSCSVMHEALHNHYTQKSLSLSPGKHHHHHH

SEQ ID NO: 161 - protein, 278 aa, Homo Sapiens
APCSRGSSWSAALDKCMDCASCRARPHSDFCLGCAIEGRMDPKSCDKTHTCPPCPAPELLGGPSVFLFPPKPKDTLMISRTPEVTCVVVDVSHEDPEVKFNWYVDGVEVHNAKTKPREEQYNSTYRVVSVLTVLHQDWLNGKEYKCKVSNKALPAPIEKTISKAKGQPREPQVYTLPPSREEMTKNQVSLTCLVKGFYPSDIAVEWESNGQPENNYKTTPPVLDSDGSFFLYSKLTVDKSRWQQGNVFSCSVMHEALHNHYTQKSLSLSPGKHHHHHH

SEQ ID NO: 162 - protein, 278 aa, Homo Sapiens
APCSRGSSWAADLDKCMDCASCRARPHSDFCLGCAIEGRMDPKSCDKTHTCPPCPAPELLGGPSVFLFPPKPKDTLMISRTPEVTCVVVDVSHEDPEVKFNWYVDGVEVHNAKTKPREEQYNSTYRVVSVLTVLHQDWLNGKEYKCKVSNKALPAPIEKTISKAKGQPREPQVYTLPPSREEMTKNQVSLTCLVKGFYPSDIAVEWESNGQPENNYKTTPPVLDSDGSFFLYSKLTVDKSRWQQGNVFSCSVMHEALHNHYTQKSLSLSPGKHHHHHH

SEQ ID NO: 163 - protein, 278 aa, Homo Sapiens
APCSRGSSASADLDKCMDCASCRARPHSDFCLGCAIEGRMDPKSCDKTHTCPPCPAPELLGGPSVFLFPPKPKDTLMISRTPEVTCVVVDVSHEDPEVKFNWYVDGVEVHNAKTKPREEQYNSTYRVVSVLTVLHQDWLNGKEYKCKVSNKALPAPIEKTISKAKGQPREPQVYTLPPSREEMTKNQVSLTCLVKGFYPSDIAVEWESNGQPENNYKTTPPVLDSDGSFFLYSKLTVDKSRWQQGNVFSCSVMHEALHNHYTQKSLSLSPGKHHHHHH

SEQ ID NO: 164 - protein, 278 aa, Homo Sapiens
APCSRGSAWSADLDKCMDCASCRARPHSDFCLGCAIEGRMDPKSCDKTHTCPPCPAPELLGGPSVFLFPPKPKDTLMISRTPEVTCVVVDVSHEDPEVKFNWYVDGVEVHNAKTKPREEQYNSTYRVVSVLTVLHQDWLNGKEYKCKVSNKALPAPIEKTISKAKGQPREPQVYTLPPSREEMTKNQVSLTCLVKGFYPSDIAVEWESNGQPENNYKTTPPVLDSDGSFFLYSKLTVDKSRWQQGNVFSCSVMHEALHNHYTQKSLSLSPGKHHHHHH

SEQ ID NO: 165 - protein, 278 aa, Homo Sapiens
APCSRGASWSADLDKCMDCASCRARPHSDFCLGCAIEGRMDPKSCDKTHTCPPCPAPELLGGPSVFLFPPKPKDTLMISRTPEVTCVVVDVSHEDPEVKFNWYVDGVEVHNAKTKPREEQYNSTYRVVSVLTVLHQDWLNGKEYKCKVSNKALPAPIEKTISKAKGQPREPQVYTLPPSREEMTKNQVSLTCLVKGFYPSDIAVEWESNGQPENNYKTTPPVLDSDGSFFLYSKLTVDKSRWQQGNVFSCSVMHEALHNHYTQKSLSLSPGKHHHHHH

SEQ ID NO: 166 - protein, 278 aa, Homo Sapiens
APCSAGSSWSADLDKCMDCASCRARPHSDFCLGCAIEGRMDPKSCDKTHTCPPCPAPELLGGPSVFLFPPKPKDTLMISRTPEVTCVVVDVSHEDPEVKFNWYVDGVEVHNAKTKPREEQYNSTYRVVSVLTVLHQDWLNGKEYKCKVSNKALPAPIEKTISKAKGQPREPQVYTLPPSREEMTKNQVSLTCLVKGFYPSDIAVEWESNGQPENNYKTTPPVLDSDGSFFLYSKLTVDKSRWQQGNVFSCSVMHEALHNHYTQKSLSLSPGKHHHHHH

SEQ ID NO: 167 - protein, 278 aa, Homo Sapiens
APCARGSSWSADLDKCMDCASCRARPHSDFCLGCAIEGRMDPKSCDKTHTCPPCPAPELLGGPSVFLFPPKPKDTLMISRTPEVTCVVVDVSHEDPEVKFNWYVDGVEVHNAKTKPREEQYNSTYRVVSVLTVLHQDWLNGKEYKCKVSNKALPAPIEKTISKAKGQPREPQVYTLPPSREEMTKNQVSLTCLVKGFYPSDIAVEWESNGQPENNYKTTPPVLDSDGSFFLYSKLTVDKSRWQQGNVFSCSVMHEALHNHYTQKSLSLSPGKHHHHHH

SEQ ID NO: 168 - protein, 53 aa, Homo Sapiens
EQAPGTAPCSRGSSWSADLDKCMDCASCRARPHSDFCLGCAAAPPAPFRLLWP

SEQ ID NO: 169 - protein, 129 aa, Homo Sapiens
MARGSLRRLLRLLVLGLWLALLRSVAGEQAPGTAPCSRGSSWSADLDKCMDCASCRARPHSDFCLGCAAAPPAPFRLLWPILGGALSLTFVLGLLSGFLVWRRCRRREKFTTPIEETGGEGCPAVALIQ

SEQ ID NO: 170 - DNA, 959 bp, Homo Sapiens
  source 1..959: mol_type = unassigned DNA
atggctcggggctcgctgcgccggttgctgcggctcctcgtgctggggctctggctggcgttgctgcgctccgtggccggggagcaagcgccaggcaccgccccctgctcccgcggcagctcctggagcgcggacctggacaagtgcatggactgcgcgtcttgcagggcgcgaccgcacagcgacttctgcctgggctgcgctgcagcacctcctgcccccttccggctgctttggcccatccttgggggcgctctgagcctgaccttcgtgctggggctgctttctggctttttggtctggagacgatgccgcaggagagagaagttcaccacccccatagaggagaccggcggagagggctgcccagctgtggcgctgatccagtgacaatgtgccccctgccagccggggctcgcccactcatcattcattcatccattctagagccagtctctgcctcccagacgcggcgggagccaagctcctccaaccacaaggggggtggggggcggtgaatcacctctgaggcctgggcccagggttcaggggaaccttccaaggtgtctggttgccctgcctctggctccagaacagaaagggagcctcacgctggctcacacaaaacagctgacactgactaaggaactgcagcatttgcacaggggaggggggtgccctccttccttaggacctgggggccaggctgacttggggggcagacttgacactaggccccactcactcagatgtcctgaaattccaccacgggggtcaccctggggggttagggacctatttttaacactaggggctggcccactaggagggctggccctaagatacagacccccccaactccccaaagcggggaggagatatttattttggggagagtttggaggggagggagaatttattaataaaagaatctttaactttaaaaaaaaaaaaaaaaa

SEQ ID NO: 171 - protein, 5 aa, Homo Sapiens
  SITE 5: note = X can be any naturally occurring amino acid according to the ST25 standard
PYPMX

SEQ ID NO: 172 - protein, 17 aa, Homo Sapiens
  SITE 8: note = X can be any naturally occurring amino acid according to the ST25 standard
YISPSGGXTHYADSVKG

SEQ ID NO: 173 - protein, 11 aa, Homo Sapiens
GGDTYFDYFDY

SEQ ID NO: 174 - protein, 11 aa, Homo Sapiens
  SITE 8: note = X can be any naturally occurring amino acid according to the ST25 standard
RASQSISXYLN

SEQ ID NO: 175 - protein, 7 aa, Homo Sapiens
  SITE 1: note = X can be any naturally occurring amino acid according to the ST25 standard
XASSLQS

SEQ ID NO: 176 - protein, 10 aa, Homo Sapiens
  SITE 5..6: note = X can be any naturally occurring amino acid according to the ST25 standard
  SITE 8: note = X can be any naturally occurring amino acid according to the ST25 standard
QQSYXXPXIT

SEQ ID NO: 177 - DNA, 645 bp, Homo Sapiens
  source 1..645: mol_type = unassigned DNA
gacatccagatgacccagagccccagcagcctgagcgcctccgtgggcgacagagtgaccatcacctgtcgggccagccagagcatcagcggctacctgaactggtatcagcagaagcccggcaaggcccccaagctgctgatctaccaggccagctccctgcagagcggcgtgccaagcagattcagcggcagcggctccggcaccgacttcaccctgaccatcagcagcctgcagcccgaggacttcgccacctactactgccagcagagctacaccagccccttcatcaccttcggccagggcaccaaggtggaaatcaagcggaccgtggccgctcccagcgtgttcatcttcccacccagcgacgagcagctgaagtccggcacagccagcgtggtctgcctgctgaacaacttctacccccgcgaggccaaggtgcagtggaaggtggacaacgccctgcagtccggcaactcccaggaaagcgtgaccgagcaggacagcaaggactccacctacagcctgagcagcaccctgaccctgagcaaggccgactacgagaagcacaaggtgtacgcctgcgaagtgacccaccagggcctgtccagccccgtgaccaagagcttcaaccggggcgagtgc

SEQ ID NO: 178 - DNA, 1347 bp, Homo Sapiens
  source 1..1347: mol_type = unassigned DNA
gaagttcaattgttagagtccggcggaggcctggtgcagcctggcggcagcctgagactgtcttgcgccgccagcggcttcacattcagcccctaccccatgatctgggtccgccaggctccaggcaagggcctggaatgggtgtcctacatcagccccagcggcggcagcacccactacgccgatagcgtgaagggccggttcaccatcagccgggacaacagcaagaacaccctgtacctgcagatgaacagcctgcgggccgaggacaccgccgtgtactattgcgccagaggcggcgacacctacttcgattacttcgactactggggccagggcaccctggtgacagtgtccagcgcctccaccaagggcccatcggtcttcccgctagcacccagcagcaagagcaccagcggcggaacagccgccctgggctgcctggtgaaagactacttccccgagcccgtgaccgtgtcctggaactctggcgccctgaccagcggagtgcataccttccccgccgtgctgcagagcagcggcctgtacagcctgagcagcgtggtgacagtgcccagcagcagcctgggaacccagacctacatctgcaacgtgaaccacaagcccagcaacaccaaggtggacaagaaggtggaacccaagagctgcgacaagacccacacctgtcccccctgccctgcccctgaactgctgggcggacccagcgtgttcctgttccccccaaagcccaaggacaccctgatgatcagccggacccccgaagtgacctgcgtggtggtggacgtgtcccacgaggacccagaagtgaagtttaattggtacgtggacggcgtggaagtgcataacgccaagaccaagcccagagaggaacagtacaacagcacctaccgggtggtgtccgtgctgaccgtgctgcaccaggactggctgaacggcaaagagtacaagtgcaaggtctccaacaaggccctgcctgcccccatcgagaaaaccatcagcaaggccaagggccagccccgcgagcctcaggtgtacacactgccccccagccgggatgagctgaccaagaaccaggtgtccctgacctgtctggtgaaaggcttctaccccagcgatatcgccgtggaatgggagagcaacggccagcccgagaacaattacaagaccaccccccctgtgctggacagcgacggctcattcttcctgtactccaagctgaccgtggacaagagccggtggcagcagggcaacgtgttcagctgcagcgtgatgcacgaggccctgcacaatcactacacccagaagtccctgagcctgagccccggc

SEQ ID NO: 179 - DNA, 645 bp, Homo Sapiens
  source 1..645: mol_type = unassigned DNA
gacatccagatgacccagtctccagccaccctgtctgcatctgtaggagacagagtcaccatcacttgccgggcaagtcagagcattagcggctatttaaattggtatcagcagaaaccagggaaagcccctaagctcctgatctatcaggcatccagtttgcaaagtggggtcccatcaaggttcagtggcagtggatctgggacagatttcactctcaccatcagcagtctgcaacctgaagattttgcaacttactactgtcaacagagctacactagtccattcatcactttcggccctgggaccaaggtggagatcaaacgaactgtggctgcaccatctgtcttcatcttcccgccatctgatgagcagttgaaatctggaactgcctctgttgtgtgcctgctgaataacttctatcccagagaggccaaagtacagtggaaggtggataacgccctccaatcgggtaactcccaggagagtgtcacagagcaggacagcaaggacagcacctacagcctcagcagcaccctgacgctgagcaaagcagactacgagaaacacaaactctacgcctgcgaagtcacccatcagggcctgagctcgcccgtcacaaagagcttcaacaggggagagtgt

SEQ ID NO: 180 - DNA, 1347 bp, Homo Sapiens
  source 1..1347: mol_type = unassigned DNA
gaagttcaattgttagagtctggtggcggtcttgttcagcctggtggttctttacgtctttcttgcgctgcttccggattcactttctctccttaccctatgatctgggttcgccaagctcctggtaaaggtttggagtgggtttcttatatctctccttctggtggcaagactcattatgctgactccgttaaaggtcgcttcactatctctagagacaactctaagaatactctctacttgcagatgaacagcttaagggctgaggacacggccgtgtattactgtgcgagagggggtgatacttatttcgactactttgactactggggccagggaaccctggtcaccgtctcaagcgcctccaccaagggcccatcggtcttcccgctagcacccagcagcaagagcaccagcggcggaacagccgccctgggctgcctggtgaaagactacttccccgagcccgtgaccgtgtcctggaactctggcgccctgaccagcggagtgcataccttccccgccgtgctgcagagcagcggcctgtacagcctgagcagcgtggtgacagtgcccagcagcagcctgggaacccagacctacatctgcaacgtgaaccacaagcccagcaacaccaaggtggacaagaaggtggaacccaagagctgcgacaagacccacacctgtcccccctgccctgcccctgaactgctgggcggacccagcgtgttcctgttccccccaaagcccaaggacaccctgatgatcagccggacccccgaagtgacctgcgtggtggtggacgtgtcccacgaggacccagaagtgaagtttaattggtacgtggacggcgtggaagtgcataacgccaagaccaagcccagagaggaacagtacaacagcacctaccgggtggtgtccgtgctgaccgtgctgcaccaggactggctgaacggcaaagagtacaagtgcaaggtctccaacaaggccctgcctgcccccatcgagaaaaccatcagcaaggccaagggccagccccgcgagcctcaggtgtacacactgccccccagccgggatgagctgaccaagaaccaggtgtccctgacctgtctggtgaaaggcttctaccccagcgatatcgccgtggaatgggagagcaacggccagcccgagaacaattacaagaccaccccccctgtgctggacagcgacggctcattcttcctgtactccaagctgaccgtggacaagagccggtggcagcagggcaacgtgttcagctgcagcgtgatgcacgaggccctgcacaatcactacacccagaagtccctgagcctgagccccggc

SEQ ID NO: 181 - DNA, 645 bp, Homo Sapiens
  source 1..645: mol_type = unassigned DNA
gacatccagatgacccagagccccagcagcctgagcgcctccgtgggcgacagagtgaccatcacctgtcgggccagccagagcatcagcagctacctgaactggtatcagcagaagcccggcaaggcccccaagctgctgatctaccaggccagctccctgcagagcggcgtgccaagcagattcagcggcagcggctccggcaccgacttcaccctgaccatcagcagcctgcagcccgaggacttcgccacctactactgccagcagagctacaccagccccttcatcaccttcggccagggcaccaaggtggaaatcaagcggaccgtggccgctcccagcgtgttcatcttcccacccagcgacgagcagctgaagtccggcacagccagcgtggtctgcctgctgaacaacttctacccccgcgaggccaaggtgcagtggaaggtggacaacgccctgcagtccggcaactcccaggaaagcgtgaccgagcaggacagcaaggactccacctacagcctgagcagcaccctgaccctgagcaaggccgactacgagaagcacaaggtgtacgcctgcgaagtgacccaccagggcctgtccagccccgtgaccaagagcttcaaccggggcgagtgc

SEQ ID NO: 182 - DNA, 1347 bp, Homo Sapiens
  source 1..1347: mol_type = unassigned DNA
gaagttcaattgttagagtccggcggaggcctggtgcagcctggcggcagcctgagactgtcttgcgccgccagcggcttcacattcagcccctaccccatgatgtgggtccgccaggctccaggcaagggcctggaatgggtgtcctacatcagccccagcggcggcagcacccactacgccgatagcgtgaagggccggttcaccatcagccgggacaacagcaagaacaccctgtacctgcagatgaacagcctgcgggccgaggacaccgccgtgtactattgcgccagaggcggcgacacctacttcgattacttcgactactggggccagggcaccctggtgacagtgtccagcgcctccaccaagggcccatcggtcttcccgctagcacccagcagcaagagcaccagcggcggaacagccgccctgggctgcctggtgaaagactacttccccgagcccgtgaccgtgtcctggaactctggcgccctgaccagcggagtgcataccttccccgccgtgctgcagagcagcggcctgtacagcctgagcagcgtggtgacagtgcccagcagcagcctgggaacccagacctacatctgcaacgtgaaccacaagcccagcaacaccaaggtggacaagaaggtggaacccaagagctgcgacaagacccacacctgtcccccctgccctgcccctgaactgctgggcggacccagcgtgttcctgttccccccaaagcccaaggacaccctgatgatcagccggacccccgaagtgacctgcgtggtggtggacgtgtcccacgaggacccagaagtgaagtttaattggtacgtggacggcgtggaagtgcataacgccaagaccaagcccagagaggaacagtacaacagcacctaccgggtggtgtccgtgctgaccgtgctgcaccaggactggctgaacggcaaagagtacaagtgcaaggtctccaacaaggccctgcctgcccccatcgagaaaaccatcagcaaggccaagggccagccccgcgagcctcaggtgtacacactgccccccagccgggatgagctgaccaagaaccaggtgtccctgacctgtctggtgaaaggcttctaccccagcgatatcgccgtggaatgggagagcaacggccagcccgagaacaattacaagaccaccccccctgtgctggacagcgacggctcattcttcctgtactccaagctgaccgtggacaagagccggtggcagcagggcaacgtgttcagctgcagcgtgatgcacgaggccctgcacaatcactacacccagaagtccctgagcctgagccccggc

SEQ ID NO: 183 - DNA, 645 bp, Homo Sapiens
  source 1..645: mol_type = unassigned DNA
gacatccagatgacccagtctccagccaccctgtctgcatctgtaggagacagagtcaccatcacttgccgggcaagtcagagcattagcagctatttaaattggtatcagcagaaaccagggaaagcccctaagctcctgatctatcaggcatccagtttgcaaagtggggtcccatcaaggttcagtggcagtggatctgggacagatttcactctcaccatcagcagtctgcaacctgaagattttgcaacttactactgtcaacagagctacactagtccattcatcactttcggccctgggaccaaggtggagatcaaacgaactgtggctgcaccatctgtcttcatcttcccgccatctgatgagcagttgaaatctggaactgcctctgttgtgtgcctgctgaataacttctatcccagagaggccaaagtacagtggaaggtggataacgccctccaatcgggtaactcccaggagagtgtcacagagcaggacagcaaggacagcacctacagcctcagcagcaccctgacgctgagcaaagcagactacgagaaacacaaactctacgcctgcgaagtcacccatcagggcctgagctcgcccgtcacaaagagcttcaacaggggagagtgt

SEQ ID NO: 184 - DNA, 1347 bp, Homo Sapiens
  source 1..1347: mol_type = unassigned DNA
gaagttcaattgttagagtctggtggcggtcttgttcagcctggtggttctttacgtctttcttgcgctgcttccggattcactttctctccttaccctatgatgtgggttcgccaagctcctggtaaaggtttggagtgggtttcttatatctctccttctggtggcaagactcattatgctgactccgttaaaggtcgcttcactatctctagagacaactctaagaatactctctacttgcagatgaacagcttaagggctgaggacacggccgtgtattactgtgcgagagggggtgatacttatttcgactactttgactactggggccagggaaccctggtcaccgtctcaagcgcctccaccaagggcccatcggtcttcccgctagcacccagcagcaagagcaccagcggcggaacagccgccctgggctgcctggtgaaagactacttccccgagcccgtgaccgtgtcctggaactctggcgccctgaccagcggagtgcataccttccccgccgtgctgcagagcagcggcctgtacagcctgagcagcgtggtgacagtgcccagcagcagcctgggaacccagacctacatctgcaacgtgaaccacaagcccagcaacaccaaggtggacaagaaggtggaacccaagagctgcgacaagacccacacctgtcccccctgccctgcccctgaactgctgggcggacccagcgtgttcctgttccccccaaagcccaaggacaccctgatgatcagccggacccccgaagtgacctgcgtggtggtggacgtgtcccacgaggacccagaagtgaagtttaattggtacgtggacggcgtggaagtgcataacgccaagaccaagcccagagaggaacagtacaacagcacctaccgggtggtgtccgtgctgaccgtgctgcaccaggactggctgaacggcaaagagtacaagtgcaaggtctccaacaaggccctgcctgcccccatcgagaaaaccatcagcaaggccaagggccagccccgcgagcctcaggtgtacacactgccccccagccgggatgagctgaccaagaaccaggtgtccctgacctgtctggtgaaaggcttctaccccagcgatatcgccgtggaatgggagagcaacggccagcccgagaacaattacaagaccaccccccctgtgctggacagcgacggctcattcttcctgtactccaagctgaccgtggacaagagccggtggcagcagggcaacgtgttcagctgcagcgtgatgcacgaggccctgcacaatcactacacccagaagtccctgagcctgagccccggc

SEQ ID NO: 185 - DNA, 645 bp, Homo Sapiens
  source 1..645: mol_type = unassigned DNA
gacatccagatgacccagagccccagcagcctgtctgccagcgtgggcgacagagtgaccatcacctgtagagccagccagagcatcagcagctacctgaactggtatcagcagaagcccggcaaggcccccaagctgctgatctatgccgccagctctctgcagagcggagtgcccagcagattttctggcagcggcagcggcaccgacttcaccctgacaatcagcagcctgcagcccgaggacttcgccacctactactgccagcagagctacagcacccccggcatcacatttggccagggcaccaaggtggaaatcaagcggacagtggccgctcccagcgtgttcatcttcccacctagcgacgagcagctgaagtccggcacagccagcgtcgtgtgcctgctgaacaacttctacccccgcgaggccaaggtgcagtggaaggtggacaatgccctgcagtccggcaactcccaggaaagcgtcaccgagcaggacagcaaggactccacctacagcctgagcagcaccctgaccctgagcaaggccgactacgagaagcacaaggtgtacgcctgcgaagtgacccaccagggcctgtctagccccgtgaccaagagcttcaaccggggcgagtgt

SEQ ID NO: 186 - DNA, 1347 bp, Homo Sapiens
  source 1..1347: mol_type = unassigned DNA
gaagttcaattgttagagtccggcggaggcctggtgcagcctggcggatctctgagactgagctgtgccgccagcggcttcaccttcagcccctaccctatgatgtgggtccgacaggcccctggcaagggactggaatgggtgtcctacatctctcccagcggcggcagcacccactacgccgattctgtgaagggccggttcaccatcagccgggacaacagcaagaacaccctgtacctgcagatgaacagcctgcgggccgaggacaccgccgtgtactattgtgccagaggcggcgacacctacttcgattacttcgactactggggccagggcaccctggtcaccgtgtcatctgcctccaccaagggcccatcggtcttcccgctagcacccagcagcaagagcaccagcggcggaacagccgccctgggctgcctggtgaaagactacttccccgagcccgtgaccgtgtcctggaactctggcgccctgaccagcggagtgcataccttccccgccgtgctgcagagcagcggcctgtacagcctgagcagcgtggtgacagtgcccagcagcagcctgggaacccagacctacatctgcaacgtgaaccacaagcccagcaacaccaaggtggacaagaaggtggaacccaagagctgcgacaagacccacacctgtcccccctgccctgcccctgaactgctgggcggacccagcgtgttcctgttccccccaaagcccaaggacaccctgatgatcagccggacccccgaagtgacctgcgtggtggtggacgtgtcccacgaggacccagaagtgaagtttaattggtacgtggacggcgtggaagtgcataacgccaagaccaagcccagagaggaacagtacaacagcacctaccgggtggtgtccgtgctgaccgtgctgcaccaggactggctgaacggcaaagagtacaagtgcaaggtctccaacaaggccctgcctgcccccatcgagaaaaccatcagcaaggccaagggccagccccgcgagcctcaggtgtacacactgccccccagccgggatgagctgaccaagaaccaggtgtccctgacctgtctggtgaaaggcttctaccccagcgatatcgccgtggaatgggagagcaacggccagcccgagaacaattacaagaccaccccccctgtgctggacagcgacggctcattcttcctgtactccaagctgaccgtggacaagagccggtggcagcagggcaacgtgttcagctgcagcgtgatgcacgaggccctgcacaatcactacacccagaagtccctgagcctgagccccggc

SEQ ID NO: 187 - DNA, 645 bp, Homo Sapiens
  source 1..645: mol_type = unassigned DNA
gacatccagatgacccagtctccagccaccctgtctgcatctgtaggagacagagtcaccatcacttgccgggcaagtcagagcattagcagctatttaaattggtatcagcagaaaccagggaaagcccctaagctcctgatctatgctgcatccagtttgcaaagtggggtcccatcaaggttcagtggcagtggatctgggacagatttcactctcaccatcagcagtctgcaacctgaagattttgcaacttactactgtcaacagagctactctagtccagggatcactttcggccctgggaccaaggtggagatcaaacgaactgtggctgcaccatctgtcttcatcttcccgccatctgatgagcagttgaaatctggaactgcctctgttgtgtgcctgctgaataacttctatcccagagaggccaaagtacagtggaaggtggataacgccctccaatcgggtaactcccaggagagtgtcacagagcaggacagcaaggacagcacctacagcctcagcagcaccctgacgctgagcaaagcagactacgagaaacacaaactctacgcctgcgaagtcacccatcagggcctgagctcgcccgtcacaaagagcttcaacaggggagagtgt

SEQ ID NO: 188 - DNA, 1347 bp, Homo Sapiens
  source 1..1347: mol_type = unassigned DNA
gaagttcaattgttagagtctggtggcggtcttgttcagcctggtggttctttacgtctttcttgcgctgcttccggattcactttctctccttaccctatgatgtgggttcgccaagctcctggtaaaggtttggagtgggtttcttatatctctccttctggtggcaagactcattatgctgactccgttaaaggtcgcttcactatctctagagacaactctaagaatactctctacttgcagatgaacagcttaagggctgaggacacggccgtgtattactgtgcgagagggggtgatacgtatttcgactactttgactactggggccagggaaccctggtcaccgtctcaagcgcctccaccaagggcccatcggtcttcccgctagcacccagcagcaagagcaccagcggcggaacagccgccctgggctgcctggtgaaagactacttccccgagcccgtgaccgtgtcctggaactctggcgccctgaccagcggagtgcataccttccccgccgtgctgcagagcagcggcctgtacagcctgagcagcgtggtgacagtgcccagcagcagcctgggaacccagacctacatctgcaacgtgaaccacaagcccagcaacaccaaggtggacaagaaggtggaacccaagagctgcgacaagacccacacctgtcccccctgccctgcccctgaactgctgggcggacccagcgtgttcctgttccccccaaagcccaaggacaccctgatgatcagccggacccccgaagtgacctgcgtggtggtggacgtgtcccacgaggacccagaagtgaagtttaattggtacgtggacggcgtggaagtgcataacgccaagaccaagcccagagaggaacagtacaacagcacctaccgggtggtgtccgtgctgaccgtgctgcaccaggactggctgaacggcaaagagtacaagtgcaaggtctccaacaaggccctgcctgcccccatcgagaaaaccatcagcaaggccaagggccagccccgcgagcctcaggtgtacacactgccccccagccgggatgagctgaccaagaaccaggtgtccctgacctgtctggtgaaaggcttctaccccagcgatatcgccgtggaatgggagagcaacggccagcccgagaacaattacaagaccaccccccctgtgctggacagcgacggctcattcttcctgtactccaagctgaccgtggacaagagccggtggcagcagggcaacgtgttcagctgcagcgtgatgcacgaggccctgcacaatcactacacccagaagtccctgagcctgagccccggc

SEQ ID NO: 189 - DNA, 651 bp, Homo Sapiens
  source 1..651: mol_type = unassigned DNA
gcacaagacatccagatgacccagtctccagccaccctgtctgcatctgtaggagacagagtcaccatcacttgccgggcaagtcagagcattagcagctatttaaattggtatcagcagaaaccagggaaagcccctaagctcctgatctatgctgcatccagtttgcaaagtggggtcccatcaaggttcagtggcagtggatctgggacagatttcactctcaccatcagcagtctgcaacctgaagattttgcaacttactactgtcaacagagctactctagtccagggatcactttcggccctgggaccaaggtggagatcaaacgaactgtggctgcaccatctgtcttcatcttcccgccatctgatgagcagttgaaatctggaactgcctctgttgtgtgcctgctgaataacttctatcccagagaggccaaagtacagtggaaggtggataacgccctccaatcgggtaactcccaggagagtgtcacagagcaggacagcaaggacagcacctacagcctcagcagcaccctgacgctgagcaaagcagactacgagaaacacaaactctacgcctgcgaagtcacccatcagggcctgagctcgcccgtcacaaagagcttcaacaggggagagtgt

SEQ ID NO: 190 - DNA, 1347 bp, Homo Sapiens
  source 1..1347: mol_type = unassigned DNA
gaagttcaattgttagagtctggtggcggtcttgttcagcctggtggttctttacgtctttcttgcgctgcttccggattcactttctctccttaccctatgatgtgggttcgccaagctcctggtaaaggtttggagtgggtttcttatatctctccttctggtggcaagactcattatgctgactccgttaaaggtcgcttcactatctctagagacaactctaagaatactctctacttgcagatgaacagcttaagggctgaggacacggccgtgtattactgtgcgagagggggtgatacgtatttcgactactttgactactggggccagggaaccctggtcaccgtctcaagcgcctccaccaagggcccatcggtcttcccgctagcacccagcagcaagagcaccagcggcggaacagccgccctgggctgcctggtgaaagactacttccccgagcccgtgaccgtgtcctggaactctggcgccctgaccagcggagtgcataccttccccgccgtgctgcagagcagcggcctgtacagcctgagcagcgtggtgacagtgcccagcagcagcctgggaacccagacctacatctgcaacgtgaaccacaagcccagcaacaccaaggtggacaagcgggtggaacccaagagctgcgacaagacccacacctgtcccccctgccctgcccctgaactgctgggcggacccagcgtgttcctgttccccccaaagcccaaggacaccctgatgatcagccggacccccgaagtgacctgcgtggtggtggacgtgtcccacgaggacccagaagtgaagtttaattggtacgtggacggcgtggaagtgcataacgccaagaccaagcccagagaggaacagtacaacagcacctaccgggtggtgtccgtgctgaccgtgctgcaccaggactggctgaacggcaaagagtacaagtgcaaggtctccaacaaggccctgcctgcccccatcgagaaaaccatcagcaaggccaagggccagccccgcgagcctcaggtgtacacactgccccccagccgggaagagatgaccaagaaccaggtgtccctgacctgtctggtgaaaggcttctaccccagcgatatcgccgtggaatgggagagcaacggccagcccgagaacaattacaagaccaccccccctgtgctggacagcgacggctcattcttcctgtactccaagctgaccgtggacaagagccggtggcagcagggcaacgtgttcagctgcagcgtgatgcacgaggccctgcacaatcactacacccagaagtccctgagcctgagccccggc

SEQ ID NO: 191 - DNA, 651 bp, Homo Sapiens; identical to SEQ ID NO: 189
  source 1..651: mol_type = unassigned DNA

SEQ ID NO: 192 - DNA, 1347 bp, Homo Sapiens
  source 1..1347: mol_type = unassigned DNA
gaagttcaattgttagagtctggtggcggtcttgttcagcctggtggttctttacgtctttcttgcgctgcttccggattcactttctctccttaccctatgatgtgggttcgccaagctcctggtaaaggtttggagtgggtttcttatatctctccttctggtggcaagactcattatgctgactccgttaaaggtcgcttcactatctctagagacaactctaagaatactctctacttgcagatgaacagcttaagggctgaggacacggccgtgtattactgtgcgagagggggtgatggttatttcgactactttgactactggggccagggaaccctggtcaccgtctcaagcgcctccaccaagggcccatcggtcttcccgctagcacccagcagcaagagcaccagcggcggaacagccgccctgggctgcctggtgaaagactacttccccgagcccgtgaccgtgtcctggaactctggcgccctgaccagcggagtgcataccttccccgccgtgctgcagagcagcggcctgtacagcctgagcagcgtggtgacagtgcccagcagcagcctgggaacccagacctacatctgcaacgtgaaccacaagcccagcaacaccaaggtggacaagcgggtggaacccaagagctgcgacaagacccacacctgtcccccctgccctgcccctgaactgctgggcggacccagcgtgttcctgttccccccaaagcccaaggacaccctgatgatcagccggacccccgaagtgacctgcgtggtggtggacgtgtcccacgaggacccagaagtgaagtttaattggtacgtggacggcgtggaagtgcataacgccaagaccaagcccagagaggaacagtacaacagcacctaccgggtggtgtccgtgctgaccgtgctgcaccaggactggctgaacggcaaagagtacaagtgcaaggtctccaacaaggccctgcctgcccccatcgagaaaaccatcagcaaggccaagggccagccccgcgagcctcaggtgtacacactgccccccagccgggaagagatgaccaagaaccaggtgtccctgacctgtctggtgaaaggcttctaccccagcgatatcgccgtggaatgggagagcaacggccagcccgagaacaattacaagaccaccccccctgtgctggacagcgacggctcattcttcctgtactccaagctgaccgtggacaagagccggtggcagcagggcaacgtgttcagctgcagcgtgatgcacgaggccctgcacaatcactacacccagaagtccctgagcctgagccccggc

SEQ ID NO: 193 - DNA, 651 bp, Homo Sapiens
  source 1..651: mol_type = unassigned DNA
gcacaagacatccagatgacccagtctccagccaccctgtctgcatctgtaggagacagagtcaccatcacttgccgggcaagtcagagcattagcggctatttaaattggtatcagcagaaaccagggaaagcccctaagctcctgatctataacgcatccagtttgcaaagtggggtcccatcaaggttcagtggcagtggatctgggacagatttcactctcaccatcagcagtctgcaacctgaagattttgcaacttactactgtcaacagagctacactagtccattcatcactttcggccctgggaccaaggtggagatcaaacgaactgtggctgcaccatctgtcttcatcttcccgccatctgatgagcagttgaaatctggaactgcctctgttgtgtgcctgctgaataacttctatcccagagaggccaaagtacagtggaaggtggataacgccctccaatcgggtaactcccaggagagtgtcacagagcaggacagcaaggacagcacctacagcctcagcagcaccctgacgctgagcaaagcagactacgagaaacacaaactctacgcctgcgaagtcacccatcagggcctgagctcgcccgtcacaaagagcttcaacaggggagagtgt

SEQ ID NO: 194 - DNA, 1347 bp, Homo Sapiens; identical to SEQ ID NO: 180
  source 1..1347: mol_type = unassigned DNA

SEQ ID NO: 195 - DNA, 651 bp, Homo Sapiens
  source 1..651: mol_type = unassigned DNA
gcacaagacatccagatgacccagtctccagccaccctgtctgcatctgtaggagacagagtcaccatcacttgccgggcaagtcagagcattagcagctatttaaattggtatcagcagaaaccagggaaagcccctaagctcctgatctataacgcatccagtttgcaaagtggggtcccatcaaggttcagtggcagtggatctgggacagatttcactctcaccatcagcagtctgcaacctgaagattttgcaacttactactgtcaacagagctacactagtccagggatcactttcggccctgggaccaaggtggagatcaaacgaactgtggctgcaccatctgtcttcatcttcccgccatctgatgagcagttgaaatctggaactgcctctgttgtgtgcctgctgaataacttctatcccagagaggccaaagtacagtggaaggtggataacgccctccaatcgggtaactcccaggagagtgtcacagagcaggacagcaaggacagcacctacagcctcagcagcaccctgacgctgagcaaagcagactacgagaaacacaaactctacgcctgcgaagtcacccatcagggcctgagctcgcccgtcacaaagagcttcaacaggggagagtgt

SEQ ID NO: 196 - DNA, 1347 bp, Homo Sapiens; identical to SEQ ID NO: 184
  source 1..1347: mol_type = unassigned DNA

SEQ ID NO: 197 - DNA, 651 bp, Homo Sapiens
  source 1..651: mol_type = unassigned DNA
gcacaagacatccagatgacccagtctccagccaccctgtctgcatctgtaggagacagagtcaccatcacttgccgggcaagtcagagcattagcggctatttaaattggtatcagcagaaaccagggaaagcccctaagctcctgatctataacgcatccagtttgcaaagtggggtcccatcaaggttcagtggcagtggatctgggacagatttcactctcaccatcagcagtctgcaacctgaagattttgcaacttactactgtcaacagagctacactagtccagggatcactttcggccctgggaccaaggtggagatcaaacgaactgtggctgcaccatctgtcttcatcttcccgccatctgatgagcagttgaaatctggaactgcctctgttgtgtgcctgctgaataacttctatcccagagaggccaaagtacagtggaaggtggataacgccctccaatcgggtaactcccaggagagtgtcacagagcaggacagcaaggacagcacctacagcctcagcagcaccctgacgctgagcaaagcagactacgagaaacacaaactctacgcctgcgaagtcacccatcagggcctgagctcgcccgtcacaaagagcttcaacaggggagagtgt

SEQ ID NO: 198 - DNA, 1347 bp, Homo Sapiens; identical to SEQ ID NO: 184
  source 1..1347: mol_type = unassigned DNA

SEQ ID NO: 199 - DNA, 651 bp, Homo Sapiens
  source 1..651: mol_type = unassigned DNA
gcacaagacatccagatgacccagtctccagccaccctgtctgcatctgtaggagacagagtcaccatcacttgccgggcaagtcagagcattagcagctatttaaattggtatcagcagaaaccagggaaagcccctaagctcctgatctataacgcatccagtttgcaaagtggggtcccatcaaggttcagtggcagtggatctgggacagatttcactctcaccatcagcagtctgcaacctgaagattttgcaacttactactgtcaacagagctacactagtccattcatcactttcggccctgggaccaaggtggagatcaaacgaactgtggctgcaccatctgtcttcatcttcccgccatctgatgagcagttgaaatctggaactgcctctgttgtgtgcctgctgaataacttctatcccagagaggccaaagtacagtggaaggtggataacgccctccaatcgggtaactcccaggagagtgtcacagagcaggacagcaaggacagcacctacagcctcagcagcaccctgacgctgagcaaagcagactacgagaaacacaaactctacgcctgcgaagtcacccatcagggcctgagctcgcccgtcacaaagagcttcaacaggggagagtgt

SEQ ID NO: 200 - DNA, 1347 bp, Homo Sapiens; identical to SEQ ID NO: 184
  source 1..1347: mol_type = unassigned DNA

SEQ ID NO: 201 - DNA, 654 bp, Mus Musculus
  source 1..654: mol_type = unassigned DNA
gatatcgtgctgacacagtctcccgccagcctggccgtgtctctcggccagagagccaccatcagctgccgggccaacaagagcgtgtccaccagcagctacagctacatgcactggtatcagcagaagcccggccagccccccaagctgctgattaagtacgccagcaacctggaaagcggcgtgcccgccagattcagcggcagcggctctggcaccgacttcatcctgaacatccaccccgtggaagaagaggacgccgccacctactactgccagcacagcagagagctgcccttcaccttcggcagcggcaccaagctggaaatcaagcgggccgatgccgcccctaccgtgtccatcttcccacccagcagcgagcagctgaccagcggcggagccagcgtcgtgtgcttcctgaacaacttctaccccaaggacatcaacgtgaagtggaagatcgacggcagcgagcggcagaacggcgtgctgaacagctggaccgaccaggacagcaaggactccacctacagcatgagcagcaccctgaccctgaccaaggacgagtacgagcggcacaacagctacacatgcgaggccacccacaagaccagcaccagccccatcgtgaagtccttcaaccggaacgagtgc

SEQ ID NO: 202 - DNA, 1350 bp, Mus Musculus
  source 1..1350: mol_type = unassigned DNA
caggtgcagctgcagcagtctggccctgaagtcgtgcggcctggcgtgtccgtgaagatcagctgcaagggcagcggctacaccttcaccgactacggcatccactgggtcaagcagagccacgccaagagcctggaatggatcggcgtgatcagcacctacaacggctacaccaactacaaccagaagttcaagggcaaggccaccatgaccgtggacaagagcagcagcaccgcctacatggaactggcccggctgaccagcgaggacagcgccatctactactgcgccagagcctactacggcaacctgtactacgccatggactactggggccagggcaccagcgtgaccgtgtcctctgccaagaccaccgcccctagcgtgtaccctctggcccctgtgtgtggcgacaccaccggcagctctgtgactctgggctgcctggtcaagggctacttccccgagcccgtgacactgacctggaacagcggcagcctgagcagcggcgtgcacacctttccagccgtgctgcagagcgacctgtacaccctgagcagctccgtgaccgtgacaagcagcacctggcccagccagagcatcacctgtaacgtggcccaccccgccagcagcaccaaggtggacaagaagatcgagcccagaggccccaccatcaagccctgccccccttgcaagtgcccagcccccaatctgctgggcggacccagcgtgttcatcttcccacccaagatcaaggacgtgctgatgatcagcctgagccccatcgtgacctgcgtggtggtggacgtgtccgaggacgaccccgacgtgcagatcagttggttcgtgaacaacgtggaagtgcacaccgcccagacccagacccacagagaggactacaacagcaccctgcgggtggtgtccgccctgcccatccagcaccaggactggatgagcggcaaagaattcaagtgcaaagtgaacaacaaggacctgcctgcccccatcgagcggaccatcagcaagcccaagggcagcgtgcgggctccccaggtgtacgtgctgcccccacccgaggaagagatgaccaagaagcaggtcacactgacctgcatggtcaccgacttcatgcccgaggacatctacgtggaatggaccaacaacggcaagaccgagctgaactacaagaacaccgagcctgtgctggacagcgacggcagctacttcatgtacagcaagctgcgggtggaaaagaaaaactgggtggaacggaacagctacagctgcagcgtggtgcacgagggcctgcacaaccaccacaccaccaagagcttcagccggacccccggc

SEQ ID NO: 203 - DNA, 654 bp, Mus Musculus
  source 1..654: mol_type = unassigned DNA
gatatcgtgctgacacagagccccgccagcctgaccgtgtctctcggccagagagccaccatcagctgccgggccagccagagcgtgtccaccagcagctacagctacatgcagtggtatcagcagcggcctggccagccccccaagctgctgattaagtacgccaccaacctggacagcggcgtgcccgccagattttctggcagcggcagcggcacagacttcaccctgaacatccaccccgtggaagaagaggacgccgccacctactactgccagcacagctgggagatcccttacaccttcggcggaggcaccaagctggaaatcaagcgggccgatgccgcccctaccgtgtccatcttcccacccagcagcgagcagctgaccagcggcggagccagcgtcgtgtgcttcctgaacaacttctaccccaaggacatcaacgtgaagtggaagatcgacggcagcgagcggcagaacggcgtgctgaacagctggaccgaccaggacagcaaggactccacctacagcatgagcagcaccctgaccctgaccaaggacgagtacgagcggcacaacagctacacatgcgaggccacccacaagaccagcaccagccccatcgtgaagtccttcaaccggaacgagtgc

SEQ ID NO: 204 - DNA, 1344 bp, Mus Musculus
  source 1..1344: mol_type = unassigned DNA
gaagtgaagctggaagagtctggcggcggactggtccagcctggcggcagcatgaagctgagctgcgtggccagcggcttcaccttcaacaactactggatgagctgggtccgacagagccccgagaagggcctggaatggctggccgagatccggctgaagtccgacaactacgccacccactacgccgagagcgtgaagggcaagttcaccatcagccgggacgacagcaagagccggctgtacctgcagatgaacaacctgcgggccgagaacaccggcatctactactgcaccggcggcttcgccgactacttcgactactggggccagggcaccaccctgaccgtgtcctctgccaagaccaccgcccctagcgtgtaccctctggcccctgtgtgtggcgacaccaccggcagctctgtgactctgggctgcctggtcaagggctacttccccgagcccgtgacactgacctggaacagcggcagcctgagcagcggcgtgcacacctttccagccgtgctgcagagcgacctgtacaccctgagcagctccgtgaccgtgacaagcagcacctggcccagccagagcatcacctgtaacgtggcccaccccgccagcagcaccaaggtggacaagaagatcgagcccagaggccccaccatcaagccctgccccccttgcaagtgcccagcccccaatctgctgggcggacccagcgtgttcatcttcccacccaagatcaaggacgtgctgatgatcagcctgagccccatcgtgacctgcgtggtggtggacgtgtccgaggacgaccccgacgtgcagatcagttggttcgtgaacaacgtggaagtgcacaccgcccagacccagacccacagagaggactacaacagcaccctgcgggtggtgtccgccctgcccatccagcaccaggactggatgagcggcaaagaattcaagtgcaaagtgaacaacaaggacctgcctgcccccatcgagcggaccatcagcaagcccaagggcagcgtgcgggctccccaggtgtacgtgctgcccccacccgaggaagagatgaccaagaagcaggtcacactgacctgcatggtcaccgacttcatgcccgaggacatctacgtggaatggaccaacaacggcaagaccgagctgaactacaagaacaccgagcctgtgctggacagcgacggcagctacttcatgtacagcaagctgcgggtggaaaagaaaaactgggtggaacggaacagctacagctgcagcgtggtgcacgagggcctgcacaaccaccacaccaccaagagcttcagccggacccccggc

SEQ ID NO: 205 - DNA, 654 bp, Homo Sapiens
  source 1..654: mol_type = unassigned DNA
gacattgtgctgacacagtctcctgcttccctggctgtatctctggggcagagggccaccatctcatgcagggccagcaaaagtgtcagtacatctagctatagttatatgcactggtaccaacagaaaccaggacagccacccaaactcctcatcaaatatgcatccaacctagaatctggggtccctgccaggttcagtggcagtgggtctgggacagacttctccctcaacatccatcccatggaggaggacgataccgcaatgtatttctgtcagcacagtagggagcttccattcacgttcggcggagggacaaagttggaaataaaacgtacggtggccgctcccagcgtgttcatcttcccacccagcgacgagcagctgaagtccggcaccgccagcgtcgtgtgcctgctgaacaacttctacccccgcgaggccaaggtgcagtggaaggtggacaacgccctgcagagcggcaacagccaggaaagcgtcaccgagcaggacagcaaggactccacctacagcctgtccagcaccctgaccctgagcaaggccgactacgagaagcacaaggtgtacgcctgcgaagtgacccaccagggcctgagcagccccgtgaccaagagcttcaaccggggcgagtgc

SEQ ID NO: 206 - DNA, 1350 bp, Homo Sapiens
  source 1..1350: mol_type = unassigned DNA
caggtccagctggtgcagtctggggctgaggtgaagaagcctggggcctcagtgaaggtttcctgcaagggttccggctacacattcactgattatggcatgcactgggtgcggcaggcccctggacaagggctagagtggatgggagttattagtacttacaatggttatacaaactacaaccagaagtttaagggcagagtcacaatgactgtagacaaatccacgagcacagcctatatggaacttcggagcttgagatctgacgatacggccgtgtattactgtgcaagagcctactatggcaacctttactatgctatggactactggggtcaaggaaccctggtcaccgtctcctcagctagcaccaaaggcccgagcgtgtttccgctggccccgagcagcaagagcaccagcggcggaacagccgccctgggctgcctggtgaaagactacttccccgaaccggtgaccgtgtcctggaactctggcgccctgaccagcggagtgcataccttccccgccgtgctgcagagcagcggcctgtacagcctgagcagcgtggtgacagtgcccagcagcagcctgggaacccagacctacatctgcaacgtgaaccacaagcccagcaacaccaaggtggacaagaaggtggaacccaagagctgcgacaagacccacacctgtcccccctgccctgcccctgaactgctgggcggacccagcgtgttcctgttccccccaaagcccaaggacaccctgatgatcagccggacccccgaagtgacctgcgtggtggtggacgtgtcccacgaggacccagaagtgaagtttaattggtacgtggacggcgtggaagtgcataacgccaagaccaagcccagagaggaacagtacaacagcacctaccgggtggtgtccgtgctgaccgtgctgcaccaggactggctgaacggcaaagagtacaagtgcaaggtctccaacaaggccctgcctgcccccatcgagaaaaccatcagcaaggccaagggccagccccgcgagcctcaggtgtacacactgccccccagccgggatgagctgaccaagaaccaggtgtccctgacctgtctggtgaaaggcttctaccccagcgatatcgccgtggaatgggagagcaacggccagcccgagaacaattacaagaccaccccccctgtgctggacagcgacggctcattcttcctgtactccaagctgaccgtggacaagagccggtggcagcagggcaacgtgttcagctgcagcgtgatgcacgaggccctgcacaatcactacacccagaagtccctgagcctgagccccggc

SEQ ID NO: 207 - DNA, 654 bp, Homo Sapiens
  source 1..654: mol_type = unassigned DNA
gatatccagatgacccagagccccagcagcctgagcgccagcgtgggcgacagagtgaccatcacctgtcgggccagccagagcgtgtccaccagcagctacagctacatgcactggtatcagcagaagcccggcaaggcccccaagctgctgattaagtacgccagcaacctggaaagcggcgtgcccagccggtttagcggctctggcagcggcaccgacttcaccctgaccatcagcagtctgcagcccgaggacttcgccacctactactgccagcacagctgggagatcccttacaccttcggcggaggcaccaaggtggaaatcaagcgtacggtggctgcaccatctgtcttcatcttcccgccatctgatgagcagttgaaatctggaactgcctctgttgtgtgcctgctgaataacttctatcccagagaggccaaagtacagtggaaggtggataacgccctccaatcgggtaactcccaggagagtgtcacagagcaggacagcaaggacagcacctacagcctcagcagcaccctgacgctgtctaaagcagactacgagaaacacaaagtctacgcctgcgaagtcacccatcagggcctgagctcgcccgtcacaaagagcttcaacaggggagagtgt

SEQ ID NO: 208 - DNA, 1347 bp, Homo Sapiens
  source 1..1347: mol_type = unassigned DNA
caggtggaattggtggaaagcggcggaggcctggtgcagcctggcggaagcctgagactgagctgtgccgccagcggcttcaccttcagcagctactggatgagctgggtccgacaggctccaggcaagggcctggaatgggtggccgagatccggctgaagtccgacaactacgccacccactacgccgagagcgtgaagggccggttcaccatcagccgggacgacagcaagaacagcctgtacctgcagatgaacagcctgcgggccgaggacaccgccgtgtactactgcaccggctactacgccgacgccatggactactggggccagggcaccctggtcaccgtcagctcagcctccaccaagggtccatcggtcttccccctggcaccctcctccaagagcacctctgggggcacagcggccctgggctgcctggtcaaggactacttccccgaaccggtgacggtgtcgtggaactcaggcgccctgaccagcggcgtgcacaccttcccggctgtcctacagtcctcaggactctactccctcagcagcgtggtgaccgtgccctccagcagcttgggcacccagacctacatctgcaacgtgaatcacaagcccagcaacaccaaggtggacaagcgggttgagcccaaatcttgtgacaaaactcacacatgcccaccgtgcccagcacctgaactcctggggggaccgtcagtcttcctcttccccccaaaacccaaggacaccctcatgatctcccggacccctgaggtcacatgcgtggtggtggacgtgagccacgaagaccctgaggtcaagttcaactggtacgtggacggcgtggaggtgcataatgccaagacaaagccgcgggaggagcagtacaacagcacgtaccgggtggtcagcgtcctcaccgtcctgcaccaggactggctgaatggcaaggagtacaagtgcaaggtctccaacaaagccctcccagcccccatcgagaaaaccatctccaaagccaaagggcagccccgagaaccacaggtgtacaccctgcccccatcccgggaagagatgaccaagaaccaggtcagcctgacctgcctggtcaaaggcttctatcccagcgacatcgccgtggagtgggagagcaatgggcagccggagaacaactacaagaccacgcctcccgtgctggactccgacggctccttcttcctctacagcaagctcaccgtggacaagagcaggtggcagcaggggaacgtcttctcatgctccgtgatgcatgaggctctgcacaaccactacacgcagaagagcctctccctgtctccgggtaaa

SEQ ID NO: 209 - DNA, 654 bp, Mus Musculus
  source 1..654: mol_type = unassigned DNA
gatatcgtgctgacacagtctcccgccagcctggccgtgtctctcggccagagagccaccatcagctgcaaggccagccagagcgtgtccaccagcacctacagctacatgcagtggtatcagcagcggcctggacagagccccaagctgctgattaagtacgccagcaagctggacagcggcgtgcccgccagattttctggcagcggcagcggcaccgacttcaccctgaacatccaccccgtggaagaagaggacaccgccacctactactgccagcacagctgggagctgccctacaccttcggcggaggcacccggctggaaatcaagagggccgatgccgcccctaccgtgtccatcttcccacccagcagcgagcagctgaccagcggcggagccagcgtcgtgtgcttcctgaacaacttctaccccaaggacatcaacgtgaagtggaagatcgacggcagcgagcggcagaacggcgtgctgaacagctggaccgaccaggacagcaaggactccacctacagcatgagcagcaccctgaccctgaccaaggacgagtacgagcggcacaacagctacacatgcgaggccacccacaagaccagcaccagccccatcgtgaagtccttcaaccggaacgagtgc

SEQ ID NO: 210 - DNA, 1344 bp, Mus Musculus
  source 1..1344: mol_type = unassigned DNA
gaagtgaagctgggagagtctggcggcggactggtccagcctggcggcagcatgaagctgagctgcgtggccagcggcttcccattcaccaaatactggatgaactgggtccgacagagccccgagaagggcctggaatgggtggccgagatccggctgaagtccgacaactacgccacccactacgccgagagcgccaagggccggttcaccatcagccgggacgacagccggtccagcgtgtacctgcagatgaacaacctgcgggccgaggacaccgccatctactactgcagccccacctatgccgacaccatggactactggggccagggcaccagcgtgacagtgtccagcgccaagaccaccgcccctagcgtgtaccctctggcccctgtgtgtggcgacaccaccggcagctctgtgactctgggctgcctggtcaagggctacttccccgagcccgtgacactgacctggaacagcggcagcctgagcagcggcgtgcacacctttccagccgtgctgcagagcgacctgtacaccctgagcagctccgtgaccgtgacaagcagcacctggcccagccagagcatcacctgtaacgtggcccaccccgccagcagcaccaaggtggacaagaagatcgagcccagaggccccaccatcaagccctgccccccttgcaagtgcccagcccccaatctgctgggcggacccagcgtgttcatcttcccacccaagatcaaggacgtgctgatgatcagcctgagccccatcgtgacctgcgtggtggtggacgtgtccgaggacgaccccgacgtgcagatcagttggttcgtgaacaacgtggaagtgcacaccgcccagacccagacccacagagaggactacaacagcaccctgcgggtggtgtccgccctgcccatccagcaccaggactggatgagcggcaaagaattcaagtgcaaagtgaacaacaaggacctgcctgcccccatcgagcggaccatcagcaagcccaagggcagcgtgcgggctccccaggtgtacgtgctgcccccacccgaggaagagatgaccaagaagcaggtcacactgacctgcatggtcaccgacttcatgcccgaggacatctacgtggaatggaccaacaacggcaagaccgagctgaactacaagaacaccgagcctgtgctggacagcgacggcagctacttcatgtacagcaagctgcgggtggaaaagaaaaactgggtggaacggaacagctacagctgcagcgtggtgcacgagggcctgcacaaccaccacaccaccaagagcttcagccggacccccggc

SEQ ID NO: 211 - DNA, 654 bp, Mus Musculus
  source 1..654: mol_type = unassigned DNA
gatatcgtgctgacacagtctcccgccagcctggccgtgtctctcggccagagagccaccatcagctgccgggccagcaagagcgtgtccaccagcagctacagctacatgcactggtatcagcagaagcccggccagccccccaagctgctgatcaagtacaccagcaacctggaaagcggcgtgcccgccagattcagcggaagcggctccggcaccgacttcatcctgaacatccaccccgtggaagaagaggacgccgccacctactactgccagcacagcagagagctgccctggaccttcggcggaggcaccaagctggaaatcaagcgggccgatgccgcccctaccgtgtccatcttcccacccagcagcgagcagctgaccagcggcggagccagcgtcgtgtgcttcctgaacaacttctaccccaaggacatcaacgtgaagtggaagatcgacggcagcgagcggcagaacggcgtgctgaacagctggaccgaccaggacagcaaggactccacctacagcatgagcagcaccctgaccctgaccaaggacgagtacgagcggcacaacagctacacatgcgaggccacccacaagaccagcaccagccccatcgtgaagtccttcaaccggaacgagtgc

SEQ ID NO: 212 - DNA, 1353 bp, Mus Musculus
  source 1..1353: mol_type = unassigned DNA
caggtgtccctgaaagagagcggccctggcatcctgcagcctagccagaccctgagcctgacctgcagcttcagcggcttcagcctgagcaccagcggcatgggcgtgtcctggatcagacagcccagcggcaagggcctggaatggctggcccacatctactgggacgacgacaagcggtacaaccccagcctgaagtcccggctgaccatctccaaggacaccagccggaatcaggtgttcctgaagatcaccagcgtggacaccgccgataccgccacctactactgcgccagaagaggccccgactactacggctactaccccatggactattggggccagggcaccagcgtgaccgtgtctgccaagaccaccgcccctagcgtgtaccctctggcccctgtgtgtggcgacaccaccggcagctctgtgactctgggctgcctggtcaagggctacttccccgagcccgtgacactgacctggaacagcggcagcctgagcagcggcgtgcacacctttccagccgtgctgcagagcgacctgtacaccctgagcagctccgtgaccgtgacaagcagcacctggcccagccagagcatcacctgtaacgtggcccaccccgccagcagcaccaaggtggacaagaagatcgagcccagaggccccaccatcaagccctgccccccttgcaagtgcccagcccccaatctgctgggcggacccagcgtgttcatcttcccacccaagatcaaggacgtgctgatgatcagcctgagccccatcgtgacctgcgtggtggtggacgtgtccgaggacgaccccgacgtgcagatcagttggttcgtgaacaacgtggaagtgcacaccgcccagacccagacccacagagaggactacaacagcaccctgcgggtggtgtccgccctgcccatccagcaccaggactggatgagcggcaaagaattcaagtgcaaagtgaacaacaaggacctgcctgcccccatcgagcggaccatcagcaagcccaagggcagcgtgcgggctccccaggtgtacgtgctgcccccacccgaggaagagatgaccaagaagcaggtcacactgacctgcatggtcaccgacttcatgcccgaggacatctacgtggaatggaccaacaacggcaagaccgagctgaactacaagaacaccgagcctgtgctggacagcgacggcagctacttcatgtacagcaagctgcgggtggaaaagaaaaactgggtggaacggaacagctacagctgcagcgtggtgcacgagggcctgcacaaccaccacaccaccaagagcttcagccggacccccggc

SEQ ID NO: 213 - protein, 1210 aa, Homo [sequence omitted]

SEQ ID NO: 214 - protein, 622 aa, Homo sapiens
MALPTARPLLGSCGTPALGSLLFLLFSLGWVQPSRTLAGETGQEAAPLDGVLANPPNISSLSPRQLLGFPCAEVSGLSTERVRELAVALAQKNVKLSTEQLRCLAHRLSEPPEDLDALPLDLLLFLNPDAFSGPQACTRFFSRITKANVDLLPRGAPERQRLLPAALACWGVRGSLLSEADVRALGGLACDLPGRFVAESAEVLLPRLVSCPGPLDQDQQEAARAALQGGGPPYGPPSTWSVSTMDALRGLLPVLGQPIIRSIPQGIVAAWRQRSSRDPSWRQPERTILRPRFRREVEKTACPSGKKAREIDESLIFYKKWELEACVDAALLATQMDRVNAIPFTYEQLDVLKHKLDELYPQGYPESVIQHLGYLFLKMSPEDIRKWNVTSLETLKALLEVNKGHEMSPQVATLIDRFVKGRGQLDKDTLDTLTAFYPGYLCSLSPEELSSVPPSSIWAVRPQDLDTCDPRQLDVLYPKARLAFQNMNGSEYFVKIQSFLGGAPTEDLKALSQQNVSMDLATFMKLRTDAVLPLTVAEVQKLLGPHVEGLKAEERHRPVRDWILRQRQDDLDTLGLGLQGGIPNGYLVLDLSMQEALSGTPCLLGPGPVLTVLALLLASTLA

SEQ ID NO: 215 - protein, 459 aa, Homo sapiens
MAPLCPSPWLPLLIPAPAPGLTVQLLLSLLLLVPVHPQRLPRMQEDSPLGGGSSGEDDPLGEEDLPSEEDSPREEDPPGEEDLPGEEDLPGEEDLPEVKPKSEEEGSLKLEDLPTVEAPGDPQEPQNNAHRDKEGDDQSHWRYGGDPPWPRVSPACAGRFQSPVDIRPQLAAFCPALRPLELLGFQLPPLPELRLRNNGHSVQLTLPPGLEMALGPGREYRALQLHLHWGAAGRPGSEHTVEGHRFPAEIHVVHLSTAFARVDEALGRPGGLAVLAAFLEEGPEENSAYEQLLSRLEEIAEEGSETQVPGLDISALLPSDFSRYFQYEGSLTTPPCAQGVIWTVFNQTVMLSAKQLHTLSDTLWGPGDSRLQLNFRATQPLNGRVIEASFPAGVDSSPRAAEPVQLNSCLAAGDILALVFGLLFAVTSVAFLVQMRRQHRRGTKGGVSYRPAEVAETGA

SEQ ID NO: 216 - protein, 346 aa, Homo sapiens [sequence omitted]

SEQ ID NO: 217 - protein, 61 aa, Homo sapiens
MKRFLFLLLTISLLVMVQIQTGLSGQNDTSQTSSPSASSNISGGIFLFFVANAIIHLFCFS

SEQ ID NO: 218 - protein, 1255 aa, Homo sapiens [sequence omitted]

SEQ ID NO: 219 - protein, 297 aa, Homo sapiens
MTTPRNSVNGTFPAEPMKGPIAMQSGPKPLFRRMSSLVGPTQSFFMRESKTLGAVQIMNGLFHIALGGLLMIPAGIYAPICVTVWYPLWGGIMYIISGSLLAATEKNSRKCLVKGKMIMNSLSLFAAISGMILSIMDILNIKISHFLKMESLNFIRAHTPYINIYNCEPANPSEKNSPSTQYCYSIQSLFLGILSVMLIFAFFQELVIAGIVENEWKRTCSRPKSNIVLLSAEEKKEQTIEIKEEVVGLTETSSQPKNEEDIEIIPIQEEEEEETETNFPEPPQDQESSPIENDSSP

SEQ ID NO: 220 - protein, 595 aa, Homo sapiens
MRVLLAALGLLFLGALRAFPQDRPFEDTCHGNPSHYYDKAVRRCCYRCPMGLFPTQQCPQRPTDCRKQCEPDYYLDEADRCTACVTCSRDDLVEKTPCAWNSSRVCECRPGMFCSTSAVNSCARCFFHSVCPAGMIVKFPGTAQKNTVCEPASPGVSPACASPENCKEPSSGTIPQAKPTPVSPATSSASTMPVRGGTRLAQEAASKLTRAPDSPSSVGRPSSDPGLSPTQPCPEGSGDCRKQCEPDYYLDEAGRCTACVSCSRDDLVEKTPCAWNSSRTCECRPGMICATSATNSRARCVPYPICAAETVTKPQDMAEKDTTFEAPPLGTQPDCNPTPENGEAPASTSPTQSLLVDSQASKTLPIPTSAPVALSSTGKPVLDAGPVLFWVILVLVVVVGSSAFLLCHRRACRKRIRQKLHLCYPVQTSQPKLELVDSRPRRSSTQLRSGASVTEPVAEERGLMSQPLMETCHSVGAAYLESLPLQDASPAGGPSSPRDLPEPRVSTEHTNNKIEKIYIMKADTVIVGTVKAELPEGRGLAGPAEPELEEELEADHTPHYPEQETEPPLGSCSDVMLSVEEEGKEDPLPTAASGK

SEQ ID NO: 221 - protein, 847 aa, Homo sapiens
MHLLGPWLLLLVLEYLAFSDSSKWVFEHPETLYAWEGACVWIPCTYRALDGDLESFILFHNPEYNKNTSKFDGTRLYESTKDGKVPSEQKRVQFLGDKNKNCTLSIHPVHLNDSGQLGLRMESKTEKWMERIHLNVSERPFPPHIQLPPEIQESQEVTLTCLLNFSCYGYPIQLQWLLEGVPMRQAAVTSTSLTIKSVFTRSELKFSPQWSHHGKIVTCQLQDADGKFLSNDTVQLNVKHTPKLEIKVTPSDAIVREGDSVTMTCEVSSSNPEYTTVSWLKDGTSLKKQNTFTLNLREVTKDQSGKYCCQVSNDVGPGRSEEVFLQVQYAPEPSTVQILHSPAVEGSQVEFLCMSLANPLPTNYTWYHNGKEMQGRTEEKVHIPKILPWHAGTYSCVAENILGTGQRGPGAELDVQYPPKKVTTVIQNPMPIREGDTVTLSCNYNSSNPSVTRYEWKPHGAWEEPSLGVLKIQNVGWDNTTIACAACNSWCSWASPVALNVQYAPRDVRVRKIKPLSEIHSGNSVSLQCDFSSSHPKEVQFFWEKNGRLLGKESQLNFDSISPEDAGSYSCWVNNSIGQTASKAWTLEVLYAPRRLRVSMSPGDQVMEGKSATLTCESDANPPVSHYTWFDWNNQSLPYHSQKLRLEPVKVQHSGAYWCQGTNSVGKGRSPLSTLTVYYSPETIGRRVAVGLGSCLAILILAICGLKLQRRWKRTQSQQGLQENSSGQSFFVRNKKVRRAPLSEGPHSLGCYNPMMEDGISYTTLRFPEMNIPRTGDAESSEMQRPPPDCDDTVTYSALHKRQVGDYENVIPDFPEDEGIHYSELIQFGVGERPQAQENVDYVILKH

SEQ ID NO: 222 - protein, 364 aa, Homo sapiens
MPLLLLLPLLWAGALAMDPNFWLQVQESVTVQEGLCVLVPCTFFHPIPYYDKNSPVHGYWFREGAIISRDSPVATNKLDQEVQEETQGRFRLLGDPSRNNCSLSIVDARRRDNGSYFFRMERGSTKYSYKSPQLSVHVTDLTHRPKILIPGTLEPGHSKNLTCSVSWACEQGTPPIFSWLSAAPTSLGPRTTHSSVLIITPRPQDHGTNLTCQVKFAGAGVTTERTIQLNVTYVPQNPTTGIFPGDGSGKQETRAGVVHGAIGGAGVTALLALCLCLIFFIVKTHRRKAARTAVGRNDTHPTTGSASPKHQKKSKLHGPTETSSCSGAAPTVEMDEELHYASLNFHGMNPSKDTSTEYSEVRTQ

SEQ ID NO: 223 - protein, 572 aa, Homo sapiens
MECLYYFLGFLLLAARLPLDAAKRFHDVLGNERPSAYMREHNQLNGWSSDENDWNEKLYPVWKRGDMRWKNSWKGGRVQAVLTSDSPALVGSNITFAVNLIFPRCQKEDANGNIVYEKNCRNEAGLSADPYVYNWTAWSEDSDGENGTGQSHHNVFPDGKPFPHHPGWRRWNFIYVFHTLGQYFQKLGRCSVRVSVNTANVTLGPQLMEVTVYRRHGRAYVPIAQVKDVYVVTDQIPVFVTMFQKNDRNSSDETFLKDLPIMFDVLIHDPSHFLNYSTINYKWSFGDNTGLFVSTNHTVNHTYVLNGTFSLNLTVKAAAPGPCPPPPPPPRPSKPTPSLATTLKSYDSNTPGPAGDNPLELSRIPDENCQINRYGHFQATITIVEGILEVNIIQMTDVLMPVPWPESSLIDFVVTCQGSIPTEVCTIISDPTCEITQNTVCSPVDVDEMCLLTVRRTFNGSGTYCVNLTLGDDTSLALTSTLISVPDRDPASPLRMANSALISVGCLAIFVTVISLLVYKKHKEYNPIENSPGNVVRSKGLSVFLNRAKAVFFPGNQEKDPLLKNQEFKGVS

SEQ ID NO: 224 - protein, 848 aa, Homo sapiens
MLQTKDLIWTLFFLGTAVSLQVDIVPSQGEISVGESKFFLCQVAGDAKDKDISWFSPNGEKLTPNQQRISVVWNDDSSSTLTIYNANIDDAGIYKCVVTGEDGSESEATVNVKIFQKLMFKNAPTPQEFREGEDAVIVCDVVSSLPPTIIWKHKGRDVILKKDVRFIVLSNNYLQIRGIKKTDEGTYRCEGRILARGEINFKDIQVIVNVPPTIQARQNIVNATANLGQSVTLVCDAEGFPEPTMSWTKDGEQIEQEEDDEKYIFSDDSSQLTIKKVDKNDEAEYICIAENKAGEQDATIHLKVFAKPKITYVENQTAMELEEQVTLTCEASGDPIPSITWRTSTRNISSEEKTLDGHMVVRSHARVSSLTLKSIQYTDAGEYICTASNTIGQDSQSMYLEVQYAPKLQGPVAVYTWEGNQVNITCEVFAYPSATISWFRDGQLLPSSNYSNIKIYNTPSASYLEVTPDSENDFGNYNCTAVNRIGQESLEFILVQADTPSSPSIDQVEPYSSTAQVQFDEPEATGGVPILKYKAEWRAVGEEVWHSKWYDAKEASMEGIVTIVGLKPETTYAVRLAALNGKGLGEISAASEFKTQPVQGEPSAPKLEGQMGEDGNSIKVNLIKQDDGGSPIRHYLVRYRALSSEWKPEIRLPSGSDHVMLKSLDWNAEYEVYVVAENQQGKSKAAHFVFRTSAQPTAIPANGSPTSGLSTGAIVGILIVIFVLLLVVVDITCYFLNKCGLFMCIAVNLCGKAGPGAKGKDMEEGKAAFSKDESKEPIVEVRTEEERTPNHDGGKHTEPNETTPLTEPEKGPVEAKPECQETETKPAPAEVKTVPNDATQTKENESKA

SEQ ID NO: 225 - protein, 193 aa, Homo sapiens
MPEEGSGCSVRRRPYGCVLRAALVPLVAGLVICLVVCIQRFAQAQQQLPLESLGWDVAELQLNHTGPQQDPRLYWQGGPALGRSFLHGPELDKGQLRIHRDGIYMVHIQVTLAICSSTTASRHHPTTLAVGICSPASRSISLLRLSFHQGCTIASQRLTPLARGDTLCTNLTGTLLPSRNTDETFFGVQWVRP

SEQ ID NO: 226 - protein, 232 aa, Homo sapiens
MHRRRSRSCREDQKPVMDDQRDLISNNEQLPMLGRRPGAPESKCSRGALYTGFSILVTLLLAGQATTAYFLYQQQGRLDKLTVTSQNLQLENLRMKLPKPPKPVSKMRMATPLLMQALPMGALPQGPMQNATKYGNMTEDHVMHLLQNADPLKVYPPLKGSFPENLRHLKNTMETIDWKVFESWMHHWLLFEMSRHSLEQKPTDAPPKESLELEDPSSGLGVTKQDLGPVPM

SEQ ID NO: 227 - protein, 557 aa, Homo sapiens
MPPPRLLFFLLFLTPMEVRPEEPLVVKVEEGDNAVLQCLKGTSDGPTQQLTWSRESPLKPFLKLSLGLPGLGIHMRPLAIWLFIFNVSQQMGGFYLCQPGPPSEKAWQPGWTVNVEGSGELFRWNVSDLGGLGCGLKNRSSEGPSSPSGKLMSPKLYVWAKDRPEIWEGEPPCLPPRDSLNQSLSQDLTMAPGSTLWLSCGVPPDSVSRGPLSWTHVHPKGPKSLLSLELKDDRPARDMWVMETGLLLPRATAQDAGKYYCHRGNLTMSFHLEITARPVLWHWLLRTGGWKVSAVTLAYLIFCLCSLVGILHLQRALVLRRKRKRMTDPTRRFFKVTPPPGSGPQNQYGNVLSLPTPTSGLGRAQRWAAGLGGTAPSYGNPSSDVQADGALGSRSPPGVGPEEEEGEGYEEPDSEEDSEFYENDSNLGQDQLSQDGSGYENPEDEPLGPEDEDSFSNAESYENEDEELTQPVARTMDFLSPHGSAWDPSREATSLAGSQSYEDMRGILYAAPQLRSIRGQPGPNHEEDADSYENMDNPDGPDPAWGGGGRMGTWSTR

SEQ ID NO: 228 - protein, 273 aa, Homo sapiens
MTPGTQSPFFLLLLLTVLTVVTGSGHASSTPGGEKETSATQRSSVPSSTEKNALSTGVSFFFLSFHISNLQFNSSLEDPSTDYYQELQRDISEMFLQIYKQGGFLGLSNIKFRPGSVVVQLTLAFREGTINVHDVETQFNQYKTEAASRYNLTISDVSVSDVPFPFSAQSGAGVPGWGIALLVLVCVLVALAIVYLIALAVCQCRRKNYGQLDIFPARDTYHPMSEYPTYHTHGRYVPPSSTDRSPYEKVSAGNGGSSLSYTNPAVAATSANL

SEQ ID NO: 229 - protein, 310 aa, Homo sapiens
MRRAALWLWLCALALSLQPALPQIVATNLPPEDQDGSGDDSDNFSGSGAGALQDITLSQQTPSTWKDTQLLTAIPTSPEPTGLEATAASTSTLPAGEGPKEGEAVVLPEVEPGLTAREQEATPRPRETTQLPTTHQASTTTATTAQEPATSHPHRDMQPGHHETSTPAGPSQADLHTPHTEDGGPSATERAAEDGASSQLPAAEGSGEQDFTFETSGENTAVVAVEPDRRNQSPVDQGATGASQGLLDRKEVLGGVIAGGLVGLIFAVCLVGFMLYRMKKKDEGSYSLEEPKQANGGAYQKPTKQEEFYA

SEQ ID NO: 230 - protein, 1048 aa, Homo sapiens
MAFPPRRRLRLGPRGLPLLLSGLLLPLCRAFNLDVDSPAEYSGPEGSYFGFAVDFFVPSASSRMFLLVGAPKANTTQPGIVEGGQVLKCDWSSTRRCQPIEFDATGNRDYAKDDPLEFKSHQWFGASVRSKQDKILACAPLYHWRTEMKQEREPVGTCFLQDGTKTVEYAPCRSQDIDADGQGFCQGGFSIDFTKADRVLLGGPGSFYWQGQLISDQVAEIVSKYDPNVYSIKYNNQLATRTAQAIFDDSYLGYSVAVGDFNGDGIDDFVSGVPRAARTLGMVYIYDGKNMSSLYNFTGEQMAAYFGFSVAATDINGDDYADVFIGAPLFMDRGSDGKLQEVGQVSVSLQRASGDFQTTKLNGFEVFARFGSAIAPLGDLDQDGFNDIAIAAPYGGEDKKGIVYIFNGRSTGLNAVPSQILEGQWAARSMPPSFGYSMKGATDIDKNGYPDLIVGAFGVDRAILYRARPVITVNAGLEVYPSILNQDNKTCSLPGTALKVSCFNVRFCLKADGKGVLPRKLNFQVELLLDKLKQKGAIRRALFLYSRSPSHSKNMTISRGGLMQCEELIAYLRDESEFRDKLTPITIFMEYRLDYRTAADTTGLQPILNQFTPANISRQAHILLDCGEDNVCKPKLEVSVDSDQKKIYIGDDNPLTLIVKAQNQGEGAYEAELIVSIPLQADFIGVVRNNEALARLSCAFKTENQTRQVVCDLGNPMKAGTQLLAGLRFSVHQQSEMDTSVKFDLQIQSSNLFDKVSPVVSHKVDLAVLAAVEIRGVSSPDHIFLPIPNWEHKENPETEEDVGPVVQHIYELRNNGPSSFSKAMLHLQWPYKYNNNTLLYILHYDIDGPMNCTSDMEINPLRIKISSLQTTEKNDTVAGQGERDHLITKRDLALSEGDIHTLGCGVAQCLKIVCQVGRLDRGKSAILYVKSLLWTETFMNKENQNHSYSLKSSASFNVIEFPYKNLPIEDITNSTLVTTNVTWGIQPAPMPVPVWVIILAVLAGLLLLAVLVFVMYRMGFFKRVRPPQEEQEREQLQPHENGEGNSET

SEQ ID NO: 231 - protein, 188 aa, Homo sapiens
MDCRKMARFSYSVIWIMAISKVFELGLVAGLGHQEFARPSRGYLAFRDDSIWPQEEPAIRPRSSQRVPPMGIQHSKELNRTCCLNGGTCMLGSFCACPPSFYGRNCEHDVRKENCGSVPHDTWLPKKCSLCKCWHGQLRCFPQAFLPGCDGLVMDEHLVASRTPELPPSARTTTFMLVGICLSIQSYY

SEQ ID NO: 232 - protein, 750 aa, Homo sapiens
MWNLLHETDSAVATARRPRWLCAGALVLAGGFFLLGFLFGWFIKSSNEATNITPKHNMKAFLDELKAENIKKFLYNFTQIPHLAGTEQNFQLAKQIQSQWKEFGLDSVELAHYDVLLSYPNKTHPNYISIINEDGNEIFNTSLFEPPPPGYENVSDIVPPFSAFSPQGMPEGDLVYVNYARTEDFFKLERDMKINCSGKIVIARYGKVFRGNKVKNAQLAGAKGVILYSDPADYFAPGVKSYPDGWNLPGGGVQRGNILNLNGAGDPLTPGYPANEYAYRRGIAEAVGLPSIPVHPIGYYDAQKLLEKMGGSAPPDSSWRGSLKVPYNVGPGFTGNFSTQKVKMHIHSTNEVTRIYNVIGTLRGAVEPDRYVILGGHRDSWVFGGIDPQSGAAVVHEIVRSFGTLKKEGWRPRRTILFASWDAEEFGLLGSTEWAEENSRLLQERGVAYINADSSIEGNYTLRVDCTPLMYSLVHNLTKELKSPDEGFEGKSLYESWTKKSPSPEFSGMPRISKLGSGNDFEVFFQRLGIASGRARYTKNWETNKFSGYPLYHSVYETYELVEKFYDPMFKYHLTVAQVRGGMVFELANSIVLPFDCRDYAVVLRKYADKIYSISMKHPQEMKTYSVSFDSLFSAVKNFTEIASKFSERLQDFDKSNPIVLRMMNDQLMFLERAFIDPLGLPDRPFYRHVIYAPSSHNKYAGESFPGIYDALFDIESKVDPSKAWGEVKRQIYVAAFTVQAAAETLSEVA

SEQ ID NO: 233 - protein, 976 aa, Homo sapiens
MELQAARACFALLWGCALAAAAAAQGKEVVLLDFAAAGGELGWLTHPYGKGWDLMQNIMNDMPIYMYSVCNVMSGDQDNWLRTNWVYRGEAERIFIELKFTVRDCNSFPGGASSCKETFNLYYAESDLDYGTNFQKRLFTKIDTIAPDEITVSSDFEARHVKLNVEERSVGPLTRKGFYLAFQDIGACVALLSVRVYYKKCPELLQGLAHFPETIAGSDAPSLATVAGTCVDHAVVPPGGEEPRMHCAVDGEWLVPIGQCLCQAGYEKVEDACQACSPGFFKFEASESPCLECPEHTLPSPEGATSCECEEGFFRAPQDPASMPCTRPPSAPHYLTAVGMGAKVELRWTPPQDSGGREDIVYSVTCEQCWPESGECGPCEASVRYSEPPHGLTRTSVTVSDLEPHMNYTFTVEARNGVSGLVTSRSFRTASVSINQTEPPKVRLEGRSTTSLSVSWSIPPPQQSRVWKYEVTYRKKGDSNSYNVRRTEGFSVTLDDLAPDTTYLVQVQALTQEGQGAGSKVHEFQTLSPEGSGNLAVIGGVAVGVVLLLVLAGVGFFIHRRRKNQRARQSPEDVYFSKSEQLKPLKTYVDPHTYEDPNQAVLKFTTEIHPSCVTRQKVIGAGEFGEVYKGMLKTSSGKKEVPVAIKTLKAGYTEKQRVDFLGEAGIMGQFSHHNIIRLEGVISKYKPMMIITEYMENGALDKFLREKDGEFSVLQLVGMLRGIAAGMKYLANMNYVHRDLAARNILVNSNLVCKVSDFGLSRVLEDDPEATYTTSGGKIPIRWTAPEAISYRKFTSASDVWSFGIVMWEVMTYGERPYWELSNHEVMKAINDGFRLPTPMDCPSAIYQLMMQCWQQERARRPKFADIVSILDKLIRAPDSLKTLADFDPRVSIRLPSTSGSEGVPFRTVSEWLESIKMQQYTEHFMAAGYTAIEKVVQMTNDDIKRIGVRLPGHQKRIAYSLLGLKDQVNTVGIPI

SEQ ID NO: 234 - protein, 668 aa, Homo sapiens
MGGKQRDEDDEAYGKPVKYDPSFRGPIKNRSCTDVICCVLFLLFILGYIVVGIVAWLYGDPRQVLYPRNSTGAYCGMGENKDKPYLLYFNIFSCILSSNIISVAENGLQCPTPQTVITSLQQELCPSFLLPSAPALGRCFPWTNVTPPALPGITNDTTIQQGISGLIDSLNARDISVKIFEDFAQSWYWILVALGVALVLSLLFILLLRLVAGPLVLVLILGVLGVLAYGIYYCWEEYRVLRDKGASISQLGFTTNLSAYQSVQETWLAALIVLAVLEAILLLMLIFLRQRIRIAIALLKEASKAVGQMMSTMFYPLVTFVLLLICIAYWAMTALYLATSGQPQYVLWASNISSPGCEKVPINTSCNPTAHLVNSSCPGLMCVFQGYSSKGLIQRSVFNLQIYGVLGLFWTLNWVLALGQCVLAGAFASFYWAFHKPQDIPTFPLISAFIRTLRYHTGSLAFGALILTLVQIARVILEYIDHKLRGVQNPVARCIMCCFKCCLWCLEKFIKFLNRNAYIMIAIYGKNFCVSAKNAFMLLMRNIVRVVVLDKVTDLLLFFGKLLVVGGVGVLSFFFFSGRIPGLGKDFKSPHLNYYWLPIMTSILGAYVIASGFFSVFGMCVDTLFLCFLEDLERNNGSLDRPYYMSKSLLKILGKKNEAPPDNKKRKK

SEQ ID NO: 235 - protein, 214 aa, synthetic construct
  REGION 1..214: note = antibody constituent
DILLTQSPVILSVSPGERVSFSCRASQSIGTNIHWYQQRTNGSPRLLIKYASESISGIPSRFSGSGSGTDFTLSINSVESEDIADYYCQQNNNWPTTFGAGTKLELKRTVAAPSVFIFPPSDEQLKSGTASVVCLLNNFYPREAKVQWKVDNALQSGNSQESVTEQDSKDSTYSLSSTLTLSKADYEKHKVYACEVTHQGLSSPVTKSFNRGEC

SEQ ID NO: 236 - protein, 449 aa, synthetic construct
  REGION 1..449: note = antibody consituent
QVQLKQSGPGLVQPSQSLSITCTVSGFSLTNYGVHWVRQSPGKGLEWLGVIWSGGNTDYNTPFTSRLSINKDNSKSQVFFKMNSLQSNDTAIYYCARALTYYDYEFAYWGQGTLVTVSAASTKGPSVFPLAPSSKSTSGGTAALGCLVKDYFPEPVTVSWNSGALTSGVHTFPAVLQSSGLYSLSSVVTVPSSSLGTQTYICNVNHKPSNTKVDKRVEPKSCDKTHTCPPCPAPELLGGPSVFLFPPKPKDTLMISRTPEVTCVVVDVSHEDPEVKFNWYVDGVEVHNAKTKPREEQYNSTYRVVSVLTVLHQDWLNGKEYKCKVSNKALPAPIEKTISKAKGQPREPQVYTLPPSREEMTKNQVSLTCLVKGFYPSDIAVEWESNGQPENNYKTTPPVLDSDGSFFLYSKLTVDKSRWQQGNVFSCSVMHEALHNHYTQKSLSLSPGK

SEQ ID NO: 237 - protein, 214 aa, synthetic construct
  REGION 1..214: note = antibody constituent
DIQMTQSPSSLSASVGDRVTITCQASQDISNYLNWYQQKPGKAPKLLIYDASNLETGVPSRFSGSGSGTDFTFTISSLQPEDIATYFCQHFDHLPLAFGGGTKVEIKRTVAAPSVFIFPPSDEQLKSGTASVVCLLNNFYPREAKVQWKVDNALQSGNSQESVTEQDSKDSTYSLSSTLTLSKADYEKHKVYACEVTHQGLSSPVTKSFNRGEC

SEQ ID NO: 238 - protein, 444 aa, synthetic construct
  REGION 1..444: note = antibody constituent
QVQLQESGPGLVKPSETLSLTCTVSGGSVSSGDYYWTWIRQSPGKGLEWIGHIYYSGNTNYNPSLKSRLTISIDTSKTQFSLKLSSVTAADTAIYYCVRDRVTGAFDIWGQGTMVTVSSASTKGPSVFPLAPCSRSTSESTAALGCLVKDYFPEPVTVSWNSGALTSGVHTFPAVLQSSGLYSLSSVVTVPSSNFGTQTYTCNVDHKPSNTKVDKTVERKCCVECPPCPAPPVAGPSVFLFPPKPKDTLMISRTPEVTCVVVDVSHEDPEVQFNWYVDGVEVHNAKTKPREEQFNSTFRVVSVLTVVHQDWLNGKEYKCKVSNKGLPAPIEKTISKTKGQPREPQVYTLPPSREEMTKNQVSLTCLVKGFYPSDIAVEWESNGQPENNYKTTPPMLDSDGSFFLYSKLTVDKSRWQQGNVFSCSVMHEALHNHYTQKSLSLSPG

SEQ ID NO: 239 - protein, 219 aa, synthetic construct
  REGION 1..219: note = antibody constituent
DIQMTQSPSSLSASVGDRVTITCRSSQNIVHSNGNTYLDWYQQTPGKAPKLLIYKVSNRFSGVPSRFSGSGSGTDFTFTISSLQPEDIATYYCFQYSHVPWTFGQGTKLQITRTVAAPSVFIFPPSDEQLKSGTASVVCLLNNFYPREAKVQWKVDNALQSGNSQESVTEQDSKDSTYSLSSTLTLSKADYEKHKVYACEVTHQGLSSPVTKSFNRGEC

SEQ ID NO: 240 - protein, 453 aa, synthetic construct
  REGION 1..453: note = antibody constituent
QVQLQQSGAEVKKPGSSVKVSCKASGYTFTNYYIYWVRQAPGQGLEWIGGINPTSGGSNFNEKFKTRVTITADESSTTAYMELSSLRSEDTAFYFCTRQGLWFDSDGRGFDFWGQGTTVTVSSASTKGPSVFPLAPSSKSTSGGTAALGCLVKDYFPEPVTVSWNSGALTSGVHTFPAVLQSSGLYSLSSVVTVPSSSLGTQTYICNVNHKPSNTKVDKKVEPKSCDKTHTCPPCPAPELLGGPSVFLFPPKPKDTLMISRTPEVTCVVVDVSHEDPEVKFNWYVDGVEVHNAKTKPREEQYNSTYRVVSVLTVLHQDWLNGKEYKCKVSNKALPAPIEKTISKAKGQPREPQVYTLPPSRDELTKNQVSLTCLVKGFYPSDIAVEWESNGQPENNYKTTPPVLDSDGSFFLYSKLTVDKSRWQQGNVFSCSVMHEALHNHYTQKSLSLSPGK

SEQ ID NO: 241 - protein, 449 aa, synthetic construct
  REGION 1..449: note = antibody constituent
EVQLLESGGGLVQPGGSLRLSCAASGFTFSPYPMIWVRQAPGKGLEWVSYISPSGGSTHYADSVKGRFTISRDNSKNTLYLQMNSLRAEDTAVYYCARGGDTYFDYFDYWGQGTLVTVSSASTKGPSVFPLAPSSKSTSGGTAALGCLVKDYFPEPVTVSWNSGALTSGVHTFPAVLQSSGLYSLSSVVTVPSSSLGTQTYICNVNHKPSNTKVDKKVEPKSCDKTHTCPPCPAPELLGGPSVFLFPPKPKDTLMISRTPEVTCVVVDVSHEDPEVKFNWYVDGVEVHNAKTKPREEQYASTYRVVSVLTVLHQDWLNGKEYKCKVSNKALPAPIEKTISKAKGQPREPQVYTLPPSRDELTKNQVSLTCLVKGFYPSDIAVEWESNGQPENNYKTTPPVLDSDGSFFLYSKLTVDKSRWQQGNVFSCSVMHEALHNHYTQKSLSLSPG

SEQ ID NO: 242 - protein, 449 aa, synthetic construct
  REGION 1..449: note = antibody constituent
EVQLLESGGGLVQPGGSLRLSCAASGFTFSPYPMIWVRQAPGKGLEWVSYISPSGGSTHYADSVKGRFTISRDNSKNTLYLQMNSLRAEDTAVYYCARGGDTYFDYFDYWGQGTLVTVSSASTKGPSVFPLAPSSKSTSGGTAALGCLVKDYFPEPVTVSWNSGALTSGVHTFPAVLQSSGLYSLSSVVTVPSSSLGTQTYICNVNHKPSNTKVDKKVEPKSCDKTHTCPPCPAPELLGGPSVFLFPPKPKDTLMISRTPEVTCVVVDVSHEDPEVKFNWYVDGVEVHNAKTKPREEQYQSTYRVVSVLTVLHQDWLNGKEYKCKVSNKALPAPIEKTISKAKGQPREPQVYTLPPSRDELTKNQVSLTCLVKGFYPSDIAVEWESNGQPENNYKTTPPVLDSDGSFFLYSKLTVDKSRWQQGNVFSCSVMHEALHNHYTQKSLSLSPG

SEQ ID NO: 243 - protein, 449 aa, synthetic construct
  REGION 1..449: note = antibody constituent
EVQLLESGGGLVQPGGSLRLSCAASGFTFSPYPMIWVRQAPGKGLEWVSYISPSGGSTHYADSVKGRFTISRDNSKNTLYLQMNSLRAEDTAVYYCARGGDTYFDYFDYWGQGTLVTVSSASTKGPSVFPLAPSSKSTSGGTAALGCLVKDYFPEPVTVSWNSGALTSGVHTFPAVLQSSGLYSLSSVVTVPSSSLGTQTYICNVNHKPSNTKVDKKVEPKSCDKTHTCPPCPAPELLGGPSVFLFPPKPKDTLMISRTPEVTCVVVDVSHEDPEVKFNWYVDGVEVHNAKTKPREENYQSTYRVVSVLTVLHQDWLNGKEYKCKVSNKALPAPIEKTISKAKGQPREPQVYTLPPSRDELTKNQVSLTCLVKGFYPSDIAVEWESNGQPENNYKTTPPVLDSDGSFFLYSKLTVDKSRWQQGNVFSCSVMHEALHNHYTQKSLSLSPG

SEQ ID NO: 244 - protein, 449 aa, synthetic construct
  REGION 1..449: note = antibody constituent
EVQLVESGGGLVQPGGSLRLSCAASGFNIKDTYIHWVRQAPGKGLEWVARIYPTNGYTRYADSVKGRFTISADTSKNTAYLQMNSLRAEDTAVYYCSRWGGDGFYAMDYWGQGTLVTVSSASTKGPSVFPLAPSSKSTSGGTAALGCLVKDYFPEPVTVSWNSGALTSGVHTFPAVLQSSGLYSLSSVVTVPSSSLGTQTYICNVNHKPSNTKVDKKVEPKSCDKTHTCPPCPAPELLGGPSVFLFPPKPKDTLMISRTPEVTCVVVDVSHEDPEVKFNWYVDGVEVHNAKTKPREEQYASTYRVVSVLTVLHQDWLNGKEYKCKVSNKALPAPIEKTISKAKGQPREPQVYTLPPSRDELTKNQVSLTCLVKGFYPSDIAVEWESNGQPENNYKTTPPVLDSDGSFFLYSKLTVDKSRWQQGNVFSCSVMHEALHNHYTQKSLSLSPG

SEQ ID NO: 245 - protein, 449 aa, synthetic construct
  REGION 1..449: note = antibody constituent
EVQLVESGGGLVQPGGSLRLSCAASGFNIKDTYIHWVRQAPGKGLEWVARIYPTNGYTRYADSVKGRFTISADTSKNTAYLQMNSLRAEDTAVYYCSRWGGDGFYAMDYWGQGTLVTVSSASTKGPSVFPLAPSSKSTSGGTAALGCLVKDYFPEPVTVSWNSGALTSGVHTFPAVLQSSGLYSLSSVVTVPSSSLGTQTYICNVNHKPSNTKVDKKVEPKSCDKTHTCPPCPAPELLGGPSVFLFPPKPKDTLMISRTPEVTCVVVDVSHEDPEVKFNWYVDGVEVHNAKTKPREEQYQSTYRVVSVLTVLHQDWLNGKEYKCKVSNKALPAPIEKTISKAKGQPREPQVYTLPPSRDELTKNQVSLTCLVKGFYPSDIAVEWESNGQPENNYKTTPPVLDSDGSFFLYSKLTVDKSRWQQGNVFSCSVMHEALHNHYTQKSLSLSPG